European Patent Specification EP 3 784 692 B1, published August 27, 2025. Title: Glucagon Like Peptide 1 (GLP-1) Fusion Peptide Coupled Cyclic Peptide Tyrosine Tyrosine Conjugates and Uses Thereof. Applicant: Janssen Pharmaceutica N.V. The sequence listing filed with the application follows.

SEQUENCE LISTING (274 sequences)

SEQ ID NO: 1 - protein, 35 aa, Artificial Sequence
  Cyclic PYY Peptide Compound
  Ala (1)..(1): Ala, wherein the Ala is a beta-alanine with a cyclic modification
  Lys (10)..(10): Lys with a PEG12-AcBr chemical modification
  Cys (30)..(30): Cys, wherein Cys is a homocysteine with a cyclic modification
  Arg (34)..(34): Arg with a psi-(R35, Y36) chemical modification
  Tyr (35)..(35): Tyr with a psi-(R35, Y36) chemical modification
AIKPEAPGEKASPEELNRYYASLRHYLNLCTRQRY

SEQ ID NO: 2 - protein, 34 aa, Artificial Sequence
  Cyclic PYY Peptide Compound
  Ile (1)..(1): Ile with a cyclic modification
  Lys (9)..(9): Lys with a AcBr chemical modification
  Leu (29)..(29): Leu, wherien Leu is a norleucine with a cyclic modification
  Arg (33)..(33): Arg with a N-Me chemical modification
IKPEAPGEKASPEELNRYYASLRHYLNLLTRQRY

SEQ ID NO: 3 - protein, 34 aa, Artificial Sequence; identical to SEQ ID NO: 2
  Cyclic PYY Peptide Compound
  Ile (1)..(1): Ile with a cyclic modification
  Lys (9)..(9): Lys with a AcBr chemical modification
  Leu (29)..(29): Leu, wherein leu is a norleucine with a cyclic modification
  Arg (33)..(33): Arg with a psi-(R35, Y36) chemical modification
  Tyr (34)..(34): Tyr with a psi-(R35, Y36) chemical modification

SEQ ID NO: 4 - protein, 35 aa, Artificial Sequence
  Cyclic PYY Peptide Compound
  Gly (1)..(1): Gly with a cyclic modification
  Lys (10)..(10): Lys with a AcBr chemical modification
  Glu (30)..(30): Glu with a cyclic modification
  Arg (34)..(34): Arg with a psi-(R35, Y36) chemical modification
  Tyr (35)..(35): Tyr with a psi-(R35, Y36) chemical modification
GISPEAPGEKASPEELNRYYASLRHYLNLETRQRY

SEQ ID NO: 5 - protein, 35 aa, Artificial Sequence; identical to SEQ ID NO: 1
  Cyclic PYY Peptide Compound
  Ala (1)..(1): Ala, wherein the alanine is a beta-alanine with a cyclic modification
  Lys (10)..(10): Lys with a PEG6-AcBr chemical modification
  Cys (30)..(30): Cys, wherein the cys is a homocysteine with a cyclic modification
  Arg (34)..(34): Arg with a psi-(R35, Y36) chemical modification
  Tyr (35)..(35): Tyr with a psi-(R35, Y36) chemical modification

SEQ ID NO: 6 - protein, 35 aa, Artificial Sequence; identical to SEQ ID NO: 1
  Cyclic PYY Peptide Compound
  Ala (1)..(1): Ala, wherein the alanine is a beta-alanine with a cyclic modification
  Lys (10)..(10): Lys with a AcBr chemical modification
  Cys (30)..(30): Cys, wherein the cys is a homocysteine with a cyclic modification
  Arg (34)..(34): Arg with a psi-(R35, Y36) chemical modification
  Tyr (35)..(35): Tyr with a psi-(R35, Y36) chemical modification

SEQ ID NO: 7 - protein, 34 aa, Artificial Sequence
  Cyclic PYY Peptide Compound
  Ile (1)..(1): Ile with a cyclic modification
  Lys (9)..(9): Lys with a PEG12-AcBr chemical modification
  Cys (29)..(29): Cys with a cyclic modification
  Arg (33)..(33): Arg with a psi-(R35, Y36) chemical modification
  Tyr (34)..(34): Tyr with a psi-(R35, Y36) chemical modification
IKPEAPGEKASPEELNRYYASLRHYLNLCTRQRY

SEQ ID NO: 8 - protein, 35 aa, Artificial Sequence; identical to SEQ ID NO: 1
  Cyclic PYY Peptide Compound
  Ala (1)..(1): Ala, wherein the alanine is a beta-alanine with a cyclic modification
  Lys (10)..(10): Lys with a PEG12-AcBr chemical modification
  Cys (30)..(30): Cys, wherein the cys is a homocysteine with a cyclic modification
  Gln (33)..(33): Gln with a N-Me chemical modification
  Arg (34)..(34): Arg with a psi-(R35, Y36) chemical modification
  Tyr (35)..(35): Tyr with a psi-(R35, Y36) chemical modification

SEQ ID NO: 9 - protein, 35 aa, Artificial Sequence; identical to SEQ ID NO: 1
  Cyclic PYY Peptide Compound
  Ala (1)..(1): Ala, wherein the alanine is a beta-alanine with a cyclic modification
  Lys (10)..(10): Lys with a PEG12-AcBr chemical modification
  Cys (30)..(30): Cys, wherein the cys is a homocysteine with a cyclic modification
  Arg (34)..(34): Arg with a N-Me and a psi-(R35, Y36) chemical modification
  Tyr (35)..(35): Tyr with a psi-(R35, Y36) chemical modification

SEQ ID NO: 10 - protein, 35 aa, Artificial Sequence
  Cyclic PYY Peptide Compound
  Ala (1)..(1): Ala, wherein the alanine is a beta-alanine with a cyclic modification
  Lys (10)..(10): Lys with a PEG12-AcBr chemical modification
  Cys (30)..(30): Cys, wherein the cys is a homocysteine with a cyclic modification
  Arg (34)..(34): Arg with a psi-(R35, Y36) chemical modification
  Tyr (35)..(35): Tyr with a psi-(R35, Y36) chemical modification
AIRPEAPGEKASPEELNRYYASLRHYLNWCTRQRY

SEQ ID NO: 11 - protein, 34 aa, Artificial Sequence
  Cyclic PYY Peptide Compound
  Ile (1)..(1): Ile with a cyclic modification
  Lys (9)..(9): Lys with a PEG12-AcBr chemical modification
  Cys (29)..(29): Cys with a cyclic modification
  Arg (33)..(33): Arg with a psi-(R35, Y36) chemical modification
  Tyr (34)..(34): Tyr with a psi-(R35, Y36) chemical modification
IRPEAPGEKASPEELNRYYASLRHYLNWCTRQRY

SEQ ID NO: 12 - protein, 33 aa, Artificial Sequence
  Cyclic PYY Peptide Compound
  Lys (1)..(1): Lys with a cyclic modification
  Lys (8)..(8): Lys with a PEG12-AcBr chemical modification
  Cys (28)..(28): Cys with a cyclic modification
  Arg (32)..(32): Arg with a psi-(R35, Y36) chemical modification
  Tyr (33)..(33): Tyr with a psi-(R35, Y36) chemical modification
KPEAPGEKASPEELNRYYASLRHYLNLCTRQRY

SEQ ID NO: 13 - protein, 35 aa, Artificial Sequence
  Cyclic PYY Peptide Compound
  Ile (1)..(1): Ile with a cyclic modification
  Lys (9)..(9): Lys with a PEG12-AcBr chemical modification
  Leu (29)..(29): Leu, wherein the leu is a norleucine with a cyclic modification
  Arg (33)..(33): Arg with a psi-(R35, Y36) chemical modification
  Tyr (34)..(34): Tyr with a psi-(R35, Y36) chemical modification
IKPEAPGEKASPEELNRYYASLRHYLNLLVTRQRY

SEQ ID NO: 14 - protein, 35 aa, Artificial Sequence
  Cyclic PYY Peptide Compound
  Ile (1)..(1): Ile with a cyclic modification
  Lys (9)..(9): Lys with a PEG-8-triazolyl-CH2CH2CO-PEG4-AcBr chemical modification
  Cys (29)..(29): Cys, wherein the cys is a homocysteine with a cyclic modification
  Arg (33)..(33): Arg with a (R35, Y36) chemical modification
  Tyr (34)..(34): Tyr with a (R35, Y36) chemical modification
IKPEAPGEKASPEELNRYYASLRHYLNLCVTRQRY

SEQ ID NO: 15 - protein, 36 aa, Artificial Sequence
  Cyclic PYY Peptide Compound
  Ala (1)..(1): Ala, wherein the alanine is a beta-alanine with a cyclic modification
  Lys (22)..(22): Lys with a PEG12-AcBr chemical modification
  Cys (30)..(30): Cys, wherein the cys is a homocysteine with a cyclic modification
  Arg (34)..(34): Arg with a psi-(R35, Y36) chemical modification
  Tyr (35)..(35): Tyr with a psi-(R35, Y36) chemical modification
AIKPEAPGEDASPEELNRYYAKLRHYLNLCVTRQRY

SEQ ID NO: 16 - protein, 36 aa, Artificial Sequence
  Cyclic PYY Peptide Compound
  Ala (1)..(1): Ala, wherein the alanine is a beta-alanine with a cyclic modification
  Lys (21)..(21): Lys with a PEG12-AcBr chemical modification
  Cys (30)..(30): Cys, wherein the cys is a homocysteine with a cyclic modification
  Arg (34)..(34): Arg with a psi-(R35, Y36) chemical modification
  Tyr (35)..(35): Tyr with a psi-(R35, Y36) chemical modification
AIKPEAPGEDASPEELNRYYKSLRHYLNLCVTRQRY

SEQ ID NO: 17 - protein, 36 aa, Artificial Sequence
  Cyclic PYY Peptide Compound
  Ala (1)..(1): Ala, wherein the alanine is a beta-alanine with a cyclic modification
  Lys (6)..(6): Lys with a PEG12-AcBr chemical modification
  Cys (30)..(30): Cys, wherein the cys is a homocysteine with a cyclic modification
  Arg (34)..(34): Arg with a psi-(R35, Y36) chemical modification
  Tyr (35)..(35): Tyr with a psi-(R35, Y36) chemical modification
AIKPEKPGEDASPEELNRYYASLRHYLNLCVTRQRY

SEQ ID NO: 18 - protein, 35 aa, Artificial Sequence
  Cyclic PYY Peptide Compound
  Gly (1)..(1): Gly with a cyclic modification
  Lys (10)..(10): Lys with a AcBr chemical modification
  Cys (29)..(29): Cys with a cyclic modification
  Arg (34)..(34): Arg with a psi-(R35, Y36) chemical modification
  Tyr (35)..(35): Tyr with a psi-(R35, Y36) chemical modification
GIKPEAPGEKASPEELNRYYASLRHYLNCVTRQRY

SEQ ID NO: 19 - protein, 35 aa, Artificial Sequence; identical to SEQ ID NO: 18
  Cyclic PYY Peptide Compound
  Gly (1)..(1): Gly with a cyclic modification
  Lys (10)..(10): Lys with a PEG12-AcBr chemical modification
  Cys (29)..(29): Cys with a cyclic modification
  Arg (34)..(34): Arg with a N-Me chemical modification

SEQ ID NO: 20 - protein, 35 aa, Artificial Sequence
  Cyclic PYY Peptide Compound
  Ala (1)..(1): Ala, wherein the alanine is a beta-alanine with a cyclic modification
  Lys (10)..(10): Lys with a PEG12-AcBr chemical modification
  Cys (29)..(29): Cys with a cyclic modification
  Arg (34)..(34): Arg with a N-Me chemical modification
AIKPEAPGEKASPEELNRYYASLRHYLNCVTRQRY

SEQ ID NO: 21 - protein, 35 aa, Artificial Sequence; identical to SEQ ID NO: 18
  Cyclic PYY Peptide Compound
  Gly (1)..(1): Gly with a cyclic modification
  Lys (10)..(10): Lys with a PEG12-AcBr chemical modification
  Cys (29)..(29): Cys, wherein the cys is a homocysteine with a cyclic modification
  Arg (34)..(34): Arg with a N-Me chemical modification

SEQ ID NO: 22 - protein, 35 aa, Artificial Sequence; identical to SEQ ID NO: 1
  Cyclic PYY Peptide Compound
  Ala (1)..(1): Ala, wherein the alanine is a beta-alanine with a cyclic modification
  Lys (10)..(10): Lys with a PEG12-AcBr chemical modification
  Cys (30)..(30): Cys, wherein the cys is a homocysteine with a cyclic modification
  Arg (34)..(34): Arg with a N-Me chemical modification

SEQ ID NO: 23 - protein, 35 aa, Artificial Sequence; identical to SEQ ID NO: 18
  Cyclic PYY Peptide Compound
  Gly (1)..(1): Gly with a cyclic modification
  Lys (10)..(10): Lys with a PEG12-AcBr chemical modification
  Cys (29)..(29): Cys, wherein the cys is a homocysteine with a cyclic modification
  Arg (34)..(34): Arg with a psi-(R35, Y36) chemical modification
  Tyr (35)..(35): Tyr with a psi-(R35, Y36) chemical modification

SEQ ID NO: 24 - protein, 35 aa, Artificial Sequence
  Cyclic PYY Peptide Compound
  Gly (1)..(1): Gly with a cyclic modification
  Lys (10)..(10): Lys with a AcBr chemical modification
  Glu (29)..(29): Glu with a cyclic modification
  Arg (34)..(34): Arg with a psi-(R35, Y36) chemical modification
  Tyr (35)..(35): Tyr with a psi-(R35, Y36) chemical modification
GISPEAPGEKASPEELNRYYASLRHYLNEVTRQRY

SEQ ID NO: 25 - protein, 35 aa, Artificial Sequence; identical to SEQ ID NO: 1
  Cyclic PYY Peptide Compound
  Ala (1)..(1): Ala, wherein the alanine is a beta-alanine with a cyclic modification
  Lys (10)..(10): Lys with a PEG24-AcBr chemical modification
  Cys (30)..(30): Cys, wherein the cys is a homocysteine with a cyclic modification
  Arg (34)..(34): Arg with a psi-(R35, Y36) chemical modification
  Tyr (35)..(35): Tyr with a psi-(R35, Y36) chemical modification

SEQ ID NO: 26 - protein, 35 aa, Artificial Sequence
  Cyclic PYY Peptide Compound
  Gly (1)..(1): Gly with a cyclic modification
  Lys (10)..(10): Lys with a AcBr chemical modification
  Cys (30)..(30): Cys, wherein the cys is a homocysteine with a cyclic modification
  Arg (34)..(34): Arg with a psi-(R35, Y36) chemical modification
  Tyr (35)..(35): Tyr with a psi-(R35, Y36) chemical modification
GIKPEAPGEKASPEELNRYYASLRHYLNLCTRQRY

SEQ ID NO: 27 - protein, 35 aa, Artificial Sequence
  Cyclic PYY Peptide Compound
  Gly (1)..(1): Gly with a cyclic modification
  Lys (10)..(10): Lys with a AcBr chemical modification
  Cys (29)..(29): Cys with a cyclic modification
  Arg (34)..(34): Arg with a N-Me chemical modification
GISPEAPGEKASPEELNRYYASLRHYLNCVTRQRY

SEQ ID NO: 28 - protein, 35 aa, Artificial Sequence; identical to SEQ ID NO: 20
  Cyclic PYY Peptide Compound
  Ala (1)..(1): Ala, wherein the alanine is a beta-alanine with a cyclic modification
  Lys (10)..(10): Lys with a AcBr chemical modification
  Cys (29)..(29): Cys with a cyclic modification
  Arg (34)..(34): Arg with a N-Me chemical modification

SEQ ID NO: 29 - protein, 35 aa, Artificial Sequence; identical to SEQ ID NO: 20
  Cyclic PYY Peptide Compound
  Ala (1)..(1): Ala, wherein the alanine is a beta-alanine with a cyclic modification
  Lys (10)..(10): Lys with a AcBr chemical modification
  Cys (29)..(29): Cys with a cyclic modification
  Arg (34)..(34): Arg with a psi-(R35, Y36) chemical modification
  Tyr (35)..(35): Tyr with a psi-(R35, Y36) chemical modification

SEQ ID NO: 30 - protein, 35 aa, Artificial Sequence; identical to SEQ ID NO: 18
  Cyclic PYY Peptide Compound
  Gly (1)..(1): Gly with a cyclic modification
  Lys (10)..(10): Lys with a AcBr chemical modification
  Cys (29)..(29): Cys with a cyclic modification
  Arg (34)..(34): Arg with a psi-(R35, Y36) chemical modification
  Tyr (35)..(35): Tyr with a psi-(R35, Y36) chemical modification

SEQ ID NO: 31 - protein, 35 aa, Artificial Sequence; identical to SEQ ID NO: 1
  Cyclic PYY Peptide Compound
  Ala (1)..(1): Ala, wherein the alanine is a beta-alanine with a cyclic modification
  Lys (10)..(10): Lys with a AcBr chemical modification
  Cys (30)..(30): Cys, wherein the cys is a homocysteine with a cyclic modification
  Arg (34)..(34): Arg with a psi-(R35, Y36) chemical modification
  Tyr (35)..(35): Tyr with a psi-(R35, Y36) chemical modification

SEQ ID NO: 32 - protein, 35 aa, Artificial Sequence; identical to SEQ ID NO: 1
  Cyclic PYY Peptide Compound
  Ala (1)..(1): Ala, wherein the alanine is a beta-alanine with a cyclic modification
  Lys (10)..(10): Lys with an AcBr chemical modification
  Cys (30)..(30): Cys, wherein the cys is a homocysteine with a cyclic modification
  Arg (34)..(34): Arg with a N-Me chemical modification

SEQ ID NO: 33 - protein, 35 aa, Artificial Sequence
  Cyclic PYY Peptide Compound
  Gly (1)..(1): Gly with a cyclic modification
  Lys (10)..(10): Lys with a AcBr chemical modification
  Glu (29)..(29): Glu with a cyclic modification
  Arg (34)..(34): Arg with a N-Me chemical modification
GIKPEAPGEDASPEELNRYYASLRHYLNEVTRQRY

SEQ ID NO: 34 - protein, 35 aa, Artificial Sequence
  Cyclic PYY Peptide Compound
  Xaa (1)..(1): Xaa is a gamma amino-butyric acid with a cyclic modification
  Lys (10)..(10): Lys with a AcBr chemical modification
  Cys (29)..(29): Cys, wherein cys is a homocysteine with a cyclic modification
  Arg (34)..(34): Arg with a N-Me chemical modification
XIKPEAPGEKASPEELNRYYASLRHYLNCVTRQRY

SEQ ID NO: 35 - protein, 34 aa, Artificial Sequence
  Cyclic PYY Peptide Compound
  Ile (1)..(1): Ile with a cyclic modification
  Lys (9)..(9): Lys with a AcBr chemical modification
  Cys (28)..(28): Cys, wherein the cys is a homocysteine with a cyclic modification
  Arg (33)..(33): Arg with a N-Me chemical modification
IKPEAPGEKASPEELNRYYASLRHYLNCVTRQRY

SEQ ID NO: 36 - protein, 34 aa, Artificial Sequence; identical to SEQ ID NO: 35
  Cyclic PYY Peptide Compound
  Ile (1)..(1): Ile with a cyclic modification
  Lys (9)..(9): Lys with a AcBr chemical modification
  Cys (28)..(28): Cys, wherein the cys is a homocysteine with a cyclic modification
  Arg (33)..(33): Arg with a psi-(R35, Y36) chemical modification
  Tyr (34)..(34): Tyr with a psi-(R35, Y36) chemical modification

SEQ ID NO: 37 - protein, 34 aa, Artificial Sequence; identical to SEQ ID NO: 35
  Cyclic PYY Peptide Compound
  Ile (1)..(1): Ile with a cyclic modification
  Lys (9)..(9): Lys with a AcBr chemical modification
  Cys (28)..(28): Cys with a cyclic modification
  Arg (33)..(33): Arg with a N-Me chemical modification

SEQ ID NO: 38 - protein, 34 aa, Artificial Sequence; identical to SEQ ID NO: 35
  Cyclic PYY Peptide Compound
  Ile (1)..(1): Ile with a cyclic modification
  Lys (9)..(9): Lys with a AcBr chemical modification
  Cys (28)..(28): Cys with a cyclic modification
  Arg (33)..(33): Arg with a psi-(R35, Y36) chemical modification
  Tyr (34)..(34): Tyr with a psi-(R35, Y36) chemical modification

SEQ ID NO: 39 - protein, 34 aa, Artificial Sequence; identical to SEQ ID NO: 35
  Cyclic PYY Peptide Compound
  Ile (1)..(1): Ile with a cyclic modification
  Lys (9)..(9): Lys with a AcBr chemical modification
  Cys (28)..(28): Cys, wherein the cys is a homocysteine with a cyclic modification
  Arg (33)..(33): Arg with a psi-(R35, Y36) chemical modification
  Tyr (34)..(34): Tyr with a psi-(R35, Y36) chemical modification

SEQ ID NO: 40 - protein, 35 aa, Artificial Sequence; identical to SEQ ID NO: 26
  Cyclic PYY Peptide Compound
  Gly (1)..(1): Gly with a cyclic modification
  Lys (10)..(10): Lys with a AcBr chemical modification
  Cys (30)..(30): Cys, wherein the cys is a homocysteine with a cyclic modification
  Arg (34)..(34): Arg with a N-Me chemical modification

SEQ ID NO: 41 - protein, 35 aa, Artificial Sequence; identical to SEQ ID NO: 26
  Cyclic PYY Peptide Compound
  Gly (1)..(1): Gly with a cyclic modification
  Lys (10)..(10): Lys with a AcBr chemical modification
  Cys (30)..(30): Cys, wherein the cys is a homocysteine with a cyclic modification
  Arg (34)..(34): Arg with a psi-(R35, Y36) chemical modification
  Tyr (35)..(35): Tyr with a psi-(R35, Y36) chemical modification

SEQ ID NO: 42 - protein, 35 aa, Artificial Sequence; identical to SEQ ID NO: 34
  Cyclic PYY Peptide Compound
  Xaa (1)..(1): Xaa is a gamma amino butyric acid with a cyclic modification
  Lys (10)..(10): Lys with a AcBr chemical modification
  Cys (29)..(29): Cys with a cyclic modification
  Arg (34)..(34): Arg with a N-Me chemical modification

SEQ ID NO: 43 - protein, 35 aa, Artificial Sequence; identical to SEQ ID NO: 34
  Cyclic PYY Peptide Compound
  Xaa (1)..(1): Xaa is a gamma amino butyric acid with a cyclic modification
  Lys (10)..(10): Lys with a AcBr chemical modification
  Cys (29)..(29): Cys with a cyclic modification
  Arg (34)..(34): Arg with a psi-(R35, Y36) chemical modification
  Tyr (35)..(35): Tyr with a psi-(R35, Y36) chemical modification

SEQ ID NO: 44 - protein, 35 aa, Artificial Sequence
  Cyclic PYY Peptide Compound
  Xaa (1)..(1): Xaa is a gamma amino butyric acid with a cyclic modification
  Lys (10)..(10): Lys with a AcBr chemical modification
  Cys (30)..(30): Cys, wherein the cys is a homocysteine with a cyclic modification
  Arg (34)..(34): Arg with a N-Me chemical modification
XIKPEAPGEKASPEELNRYYASLRHYLNLCTRQRY

SEQ ID NO: 45 - protein, 35 aa, Artificial Sequence; identical to SEQ ID NO: 44
  Cyclic PYY Peptide Compound
  Xaa (1)..(1): Xaa is a gamma amino butyric acid with a cyclic modification
  Lys (10)..(10): Lys is a AcBr chemical modification
  Cys (30)..(30): Cys, wherein the cys is a homocysteine is a cyclic modification
  Arg (34)..(34): Arg with a psi-(R35, Y36) chemical modification
  Tyr (35)..(35): Tyr with a psi-(R35, Y36) chemical modification

SEQ ID NO: 46 - protein, 35 aa, Artificial Sequence; identical to SEQ ID NO: 44
  Cyclic PYY Peptide Compound
  Xaa (1)..(1): Xaa is a gamma amino butyric acid with a cyclic modification
  Lys (10)..(10): Lys with a AcBr chemical modification
  Cys (30)..(30): Cys with a cyclic modification
  Arg (34)..(34): Arg with a N-Me chemical modification

SEQ ID NO: 47 - protein, 35 aa, Artificial Sequence; identical to SEQ ID NO: 44
  Cyclic PYY Peptide Compound
  Xaa (1)..(1): Xaa is a gamma amino butyric acid with a cyclic modification
  Lys (10)..(10): Lys with a AcBr chemical modification
  Cys (30)..(30): Cys with a cyclic modification
  Arg (34)..(34): Arg with a psi-(R35, Y36) chemical modification
  Tyr (35)..(35): Tyr with a psi-(R35, Y36) chemical modification

SEQ ID NO: 48 - protein, 35 aa, Artificial Sequence; identical to SEQ ID NO: 44
  Cyclic PYY Peptide Compound
  Xaa (1)..(1): Xaa is a delta-amino valeric acid with a cyclic modification
  Lys (10)..(10): Lys with a AcBr chemical modification
  Cys (30)..(30): Cys, wherein the cys is a homocysteine with a cyclic modification
  Arg (34)..(34): Arg with a N-Me chemical modification

SEQ ID NO: 49 - protein, 35 aa, Artificial Sequence; identical to SEQ ID NO: 44
  Cyclic PYY Peptide Compound
  Xaa (1)..(1): Xaa is a delta-amino valeric acid with a cyclic modification
  Lys (10)..(10): Lys with a AcBr chemical modification
  Cys (30)..(30): Cys, wherein the cys is a homocysteine with a cyclic modification
  Arg (34)..(34): Arg with a psi-(R35, Y36) chemical modification
  Tyr (35)..(35): Tyr with a psi-(R35, Y36) chemical modification

SEQ ID NO: 50 - protein, 35 aa, Artificial Sequence; identical to SEQ ID NO: 44
  Cyclic PYY Peptide Compound
  Xaa (1)..(1): Xaa is a delta-amino valeric acid with a cyclic modification
  Lys (10)..(10): Lys with a AcBr chemical modification
  Cys (30)..(30): Cys with a cyclic modification
  Arg (34)..(34): Arg with a N-Me chemical modification

SEQ ID NO: 51 - protein, 35 aa, Artificial Sequence; identical to SEQ ID NO: 44
  Cyclic PYY Peptide Compound
  Xaa (1)..(1): Xaa is a delta-amino valeric acid with a cyclic modification
  Lys (10)..(10): Lys with a AcBr chemical modification
  Cys (30)..(30): Cys with a cyclic modification
  Arg (34)..(34): Arg with a psi-(R35, Y36) chemical modification
  Tyr (35)..(35): Tyr with a psi-(R35, Y36) chemical modification

SEQ ID NO: 52 - protein, 35 aa, Artificial Sequence; identical to SEQ ID NO: 1
  Cyclic PYY Peptide Compound
  Ala (1)..(1): Ala, wherein the ala is a beta-alanine with a cyclic modification
  Lys (10)..(10): Lys with a AcBr chemical modification
  Cys (30)..(30): Cys with a cyclic modification
  Arg (34)..(34): Arg with a N-Me chemical modification

SEQ ID NO: 53 - protein, 35 aa, Artificial Sequence; identical to SEQ ID NO: 1
  Cyclic PYY Peptide Compound
  Ala (1)..(1): Ala, wherein the ala is a beta-alanine with a cyclic modification
  Lys (10)..(10): Lys with a AcBr chemical modification
  Cys (30)..(30): Cys with a cyclic modification
  Arg (34)..(34): Arg with a psi-(R35, Y36) chemical modification
  Tyr (35)..(35): Tyr with a psi-(R35, Y36) chemical modification

SEQ ID NO: 54 - protein, 35 aa, Artificial Sequence; identical to SEQ ID NO: 44
  Cyclic PYY Peptide Compound
  Xaa (1)..(1): Xaa is a gamma amino butyric acid with a cyclic modification
  Lys (10)..(10): Lys with a AcBr chemical modification
  Cys (30)..(30): Cys, wherein the cys is a homocysteine with a cyclic modification
  Arg (34)..(34): Arg with a psi-(R35, Y36) chemical modification
  Tyr (35)..(35): Tyr with a psi-(R35, Y36) chemical modification

SEQ ID NO: 55 - protein, 34 aa, Homo sapiens
IKPEAPGEDASPEELNRYYASLRHYLNLVTRQRY

SEQ ID NO: 56 - protein, 30 aa, Artificial Sequence
  GLP-1 (7-36)
HSEGTFTSDVSSYLEGQAAKEFIEWLVKGR

SEQ ID NO: 57 - protein, 31 aa, Artificial Sequence
  GLP-1 (7-37)
HGEGTFTSDVSSYLEEQAAKEFIAWLVKGGG

SEQ ID NO: 58 - protein, 39 aa, Artificial Sequence
  Extendin 4 (1-39)
HGEGTFTSDLSKQMEEEAVRLFIEWLKNGGPSSGAPPPS

SEQ ID NO: 59 - protein, 28 aa, Artificial Sequence
  Extendin 4 (1-28)
HGEGTFTSDLSKQMEEEAVRLFIEWLKN

SEQ ID NO: 60 - protein, 16 aa, Artificial Sequence
  Linker 1-1
GGGGAGGGGAGGGGAA

SEQ ID NO: 61 - protein, 16 aa, Artificial Sequence
  Linker 1-2
GGGGGGGGGGGGGGGA

SEQ ID NO: 62 - protein, 21 aa, Artificial Sequence
  Linker 1-3
APAPAPAPAPAPAPAPAPAPA

SEQ ID NO: 63 - protein, 25 aa, Artificial Sequence
  Linker 1-4
APAPAPAPAPAPAPAPAPAPAPAPA

SEQ ID NO: 64 - protein, 6 aa, Artificial Sequence
  Linker 1-5
APAPAP

SEQ ID NO: 65 - protein, 14 aa, Artificial Sequence
  Linker 1-6
ASAPAPAPAPAPGS

SEQ ID NO: 66 - protein, 24 aa, Artificial Sequence
  Linker 1-7
ASAPAPAPAPAPAPAPAPAPAPGS

SEQ ID NO: 67 - protein, 12 aa, Artificial Sequence
  Linker 1-8
ASGGGGSGGGGS

SEQ ID NO: 68 - protein, 22 aa, Artificial Sequence
  Linker 1-9
ASGGGGSGGGGSGGGGSGGGGS

SEQ ID NO: 69 - protein, 42 aa, Artificial Sequence
  Linker 1-10
ASGGGGSGGGGSGGGGSGGGGSGGGGSGGGGSGGGGSGGGGS

SEQ ID NO: 70 - protein, 15 aa, Artificial Sequence
  Linker 1-11
GGGGAGGGGAGGGGA

SEQ ID NO: 71 - protein, 20 aa, Artificial Sequence
  Linker 1-12
GGGGAGGGGAGGGGAGGGGA

SEQ ID NO: 72 - protein, 21 aa, Artificial Sequence
  Linker 1-13
GGGGAGGGGAGGGGAGGGGAA

SEQ ID NO: 73 - protein, 26 aa, Artificial Sequence
  Linker 1-14
GGGGAGGGGAGGGGAGGGGAGGGGAA

SEQ ID NO: 74 - protein, 6 aa, Artificial Sequence
  Linker 1-15
GGGGGG

SEQ ID NO: 75 - protein, 16 aa, Artificial Sequence
  Linker 1-16
GGGGHGGGGHGGGGHA

SEQ ID NO: 76 - protein, 21 aa, Artificial Sequence
  Linker 1-17
GGGGHGGGGHGGGGHGGGGHA

SEQ ID NO: 77 - protein, 26 aa, Artificial Sequence
  Linker 1-18
GGGGHGGGGHGGGGHGGGGHGGGGHA

SEQ ID NO: 78 - protein, 16 aa, Artificial Sequence
  Linker 1-19
GGGGPGGGGPGGGGPA

SEQ ID NO: 79 - protein, 21 aa, Artificial Sequence
  Linker 1-20
GGGGPGGGGPGGGGPGGGGPA

SEQ ID NO: 80 - protein, 26 aa, Artificial Sequence
  Linker 1-21
GGGGPGGGGPGGGGPGGGGPGGGGPA

SEQ ID NO: 81 - protein, 16 aa, Artificial Sequence
  Linker 1-22
GGGGSGGGGSGGGGSA

SEQ ID NO: 82 - protein, 21 aa, Artificial Sequence
  Linker 1-23
PAPAPAPAPAPAPAPAPAPAP

SEQ ID NO: 83 - protein, 22 aa, Artificial Sequence
  Linker 1-24
PAPAPAPAPAPAPAPAPAPAPA

SEQ ID NO: 84 - protein, 228 aa, Artificial Sequence
  Hinge-Fc Region Peptide 1
ESKYGPPCPPCPAPEAAGGPSVFLFPPKPKDTLMISRTPEVTCVVVDVSQEDPEVQFNWYVDGVEVHNAKTKPREEQFNSTYRVVSVLTVLHQDWLNGKEYKCKVSNKGLPSSIEKTISKAKGQPREPQVYTLPPSQEEMTKNQVSLTCLVKGFYPSDIAVEWESNGQPENNYKTTPPVLDSDGSFFLYSRLTVDKSRWQEGNVFSCSVMHEALHNHYTQKSLSLSLG

SEQ ID NO: 85 - protein, 224 aa, Artificial Sequence
  Hinge-Fc Region Peptide 2
GPPCPPCPAPEAAGGPSVFLFPPKPKDTLMISRTPEVTCVVVDVSQEDPEVQFNWYVDGVEVHNAKTKPREEQFNSTYRVVSVLTVLHQDWLNGKEYKCKVSNKGLPSSIEKTISKAKGQPREPQVYTLPPSQEEMTKNQVSLTCLVKGFYPSDIAVEWESNGQPENNYKTTPPVLDSDGSFFLYSRLTVDKSRWQEGNVFSCSVMHEALHNHYTQKSLSLSLG

SEQ ID NO: 86 - protein, 222 aa, Artificial Sequence
  Hinge-Fc Region Peptide 3
CPPCPAPEAAGGPSVFLFPPKPKDTLMISRTPEVTCVVVDVSQEDPEVQFNWYVDGVEVHNAKTKPREEQFNSTYRVVSVLTVLHQDWLNGKEYKCKVSNKGLPSSIEKTISKAKGQPREPQVYTLPPSQEEMTKNQVSLTCLVKGFYPSDIAVEWESNGQPENNYKTTPPVLDSDGSFFLYSRLTVDKSRWQEGNVFSCSVMHEALHNHYTQKSLSLSLGK

SEQ ID NO: 87 - protein, 221 aa, Artificial Sequence
  Hinge-Fc Region Peptide 4
CPPCPAPEAAGGPSVFLFPPKPKDTLMISRTPEVTCVVVDVSQEDPEVQFNWYVDGVEVHNAKTKPREEQFNSTYRVVSVLTVLHQDWLNGKEYKCKVSNKGLPSSIEKTISKAKGQPREPQVYTLPPSQEEMTKNQVSLTCLVKGFYPSDIAVEWESNGQPENNYKTTPPVLDSDGSFFLYSRLTVDKSRWQEGNVFSCSVMHEALHNHYTQKSLSLSLG

SEQ ID NO: 88 - protein, 225 aa, Artificial Sequence
  Hinge-Fc Region Peptide 5
GPPCPPCPAPEAAGGPSVFLFPPKPKDTLMISRTPEVTCVVVDVSQEDPEVQFNWYVDGVEVHNAKTKPREEQFNSTYRVVSVLTVLHQDWLNGKEYKCKVSNKGLPSSIEKTISKAKGQPREPQVYTLPPSQEEMTKNQVSLTCLVKGFYPSDIAVEWESNGQPENNYKTTPPVLDSDGSFFLYSRLTVDKSRWQEGNVFSCSVMHEALHNHYTQKSLSLSLGK

SEQ ID NO: 89 - protein, 229 aa, Artificial Sequence
  Hinge-Fc Region Peptide 6
ESKYGPPCPPCPAPEAAGGPSVFLFPPKPKDTLMISRTPEVTCVVVDVSQEDPEVQFNWYVDGVEVHNAKTKPREEQFNSTYRVVSVLTVLHQDWLNGKEYKCKVSNKGLPSSIEKTISKAKGQPREPQVYTLPPSQEEMTKNQVSLTCLVKGFYPSDIAVEWESNGQPENNYKTTPPVLDSDGSFFLYSRLTVDKSRWQEGNVFSCSVMHEALHNHYTQKSLSLSLGK

SEQ ID NO: 90 - protein, 228 aa, Artificial Sequence
  Hinge-Fc Region Peptide 7
ERKCCVECPPCPAPEAAGGPSVFLFPPKPKDTLMISRTPEVTCVVVDVSQEDPEVQFNWYVDGVEVHNAKTKPREEQFNSTYRVVSVLTVLHQDWLNGKEYKCKVSNKGLPSSIEKTISKAKGQPREPQVYTLPPSQEEMTKNQVSLTCLVKGFYPSDIAVEWESNGQPENNYKTTPPVLDSDGSFFLYSRLTVDKSRWQEGNVFSCSVMHEALHNHYTQKSLSLSLG

SEQ ID NO: 91 - protein, 16 aa, Artificial Sequence
  Linker 2-1
ASGSAPAPAPEEEPCA

SEQ ID NO: 92 - protein, 15 aa, Artificial Sequence
  Linker 2-2
GGGAPAPAPEEEPCA

SEQ ID NO: 93 - protein, 17 aa, Artificial Sequence
  Linker 2-3
APAPAPAPAPAPCPEEP

SEQ ID NO: 94 - protein, 14 aa, Artificial Sequence
  Linker 2-4
APAPAPAPAPAPCP

SEQ ID NO: 95 - protein, 17 aa, Artificial Sequence
  Linker 2-5
GGGGAGGGGAGGGGACA

SEQ ID NO: 96 - protein, 22 aa, Artificial Sequence
  Linker 2-6
GGGGAYCAKYDGCYGELDFWCQ

SEQ ID NO: 97 - protein, 22 aa, Artificial Sequence
  Linker 2-7
GGGGAYSAKYDGCYGELDFWGQ

SEQ ID NO: 98 - protein, 8 aa, Artificial Sequence
  Linker 2-8
AAACPEEE

SEQ ID NO: 99 - protein, 8 aa, Artificial Sequence
  Linker 2-9
AAAEEPCA

SEQ ID NO: 100 - protein, 14 aa, Artificial Sequence
  Linker 2-10
APAPAPAPCAPRRR

SEQ ID NO: 101 - protein, 9 aa, Artificial Sequence
  Linker 2-11
APAPEEPCA

SEQ ID NO: 102 - protein, 16 aa, Artificial Sequence
  Linker 2-12
ASGSAPAPAPAPCEEE

SEQ ID NO: 103 - protein, 17 aa, Artificial Sequence
  Linker 2-13
ASGSAPAPAPAPCPEEP

SEQ ID NO: 104 - protein, 14 aa, Artificial Sequence
  Linker 2-14
ASGSGGGSGGGSCA

SEQ ID NO: 105 - protein, 17 aa, Artificial Sequence
  Linker 2-15
GGGGGGGGGGGGGGGCA

SEQ ID NO: 106 - protein, 12 aa, Artificial Sequence
  Linker 2-16
GGGGSGGGGSCA

SEQ ID NO: 107 - protein, 16 aa, Artificial Sequence
  Linker 2-17
ASGSPPPPPPEPEPCA

SEQ ID NO: 108 - protein, 17 aa, Artificial Sequence
  Linker 2-18
ASGSAPAPAPAPCPEPE

SEQ ID NO: 109 - protein, 16 aa, Artificial Sequence
  Linker 2-19
ASGSGGGGSGGGGSCA

SEQ ID NO: 110 - protein, 19 aa, Artificial Sequence
  Linker 2-20
ASGSAPAPAPAPAEEEPCA

SEQ ID NO: 111 - protein, 17 aa, Artificial Sequence
  Linker 2-21
GGGGSGGGGSGGGGSCA

SEQ ID NO: 112 - protein, 20 aa, Artificial Sequence
  Linker 2-22
ASGSGGGGSGGGGSEEEACA

SEQ ID NO: 113 - protein, 289 aa, Artificial Sequence
  GLP-1 fusion 1
HGEGTFTSDVSSYLEEQAAKEFIAWLVKGGGGGGGAGGGGAGGGGAAESKYGPPCPPCPAPEAAGGPSVFLFPPKPKDTLMISRTPEVTCVVVDVSQEDPEVQFNWYVDGVEVHNAKTKPREEQFNSTYRVVSVLTVLHQDWLNGKEYKCKVSNKGLPSSIEKTISKAKGQPREPQVYTLPPSQEEMTKNQVSLTCLVKGFYPSDIAVEWESNGQPENNYKTTPPVLDSDGSFFLYSRLTVDKSRWQEGNVFSCSVMHEALHNHYTQKSLSLSLGAPAPAPAPAPAPCP

SEQ ID NO: 114 - protein, 289 aa, Artificial Sequence
  GLP-1 fusion 2
HGEGTFTSDVSSYLEEQAAKEFIAWLVKGGGGGGGGGGGGGGGGGGAESKYGPPCPPCPAPEAAGGPSVFLFPPKPKDTLMISRTPEVTCVVVDVSQEDPEVQFNWYVDGVEVHNAKTKPREEQFNSTYRVVSVLTVLHQDWLNGKEYKCKVSNKGLPSSIEKTISKAKGQPREPQVYTLPPSQEEMTKNQVSLTCLVKGFYPSDIAVEWESNGQPENNYKTTPPVLDSDGSFFLYSRLTVDKSRWQEGNVFSCSVMHEALHNHYTQKSLSLSLGAPAPAPAPAPAPCP

SEQ ID NO: 115 - protein, 294 aa, Artificial Sequence
  GLP-1 fusion 3
HGEGTFTSDVSSYLEEQAAKEFIAWLVKGGGAPAPAPAPAPAPAPAPAPAPAPAPAGPPCPPCPAPEAAGGPSVFLFPPKPKDTLMISRTPEVTCVVVDVSQEDPEVQFNWYVDGVEVHNAKTKPREEQFNSTYRVVSVLTVLHQDWLNGKEYKCKVSNKGLPSSIEKTISKAKGQPREPQVYTLPPSQEEMTKNQVSLTCLVKGFYPSDIAVEWESNGQPENNYKTTPPVLDSDGSFFLYSRLTVDKSRWQEGNVFSCSVMHEALHNHYTQKSLSLSLGAPAPAPAPAPAPCP

SEQ ID NO: 116 - protein, 286 aa, Artificial Sequence
  GLP-1 fusion 4
HGEGTFTSDLSKQMEEEAVRLFIEWLKNGGGGAGGGGAGGGGAAESKYGPPCPPCPAPEAAGGPSVFLFPPKPKDTLMISRTPEVTCVVVDVSQEDPEVQFNWYVDGVEVHNAKTKPREEQFNSTYRVVSVLTVLHQDWLNGKEYKCKVSNKGLPSSIEKTISKAKGQPREPQVYTLPPSQEEMTKNQVSLTCLVKGFYPSDIAVEWESNGQPENNYKTTPPVLDSDGSFFLYSRLTVDKSRWQEGNVFSCSVMHEALHNHYTQKSLSLSLGAPAPAPAPAPAPCP

SEQ ID NO: 117 - protein, 286 aa, Artificial Sequence
  GLP-1 fusion 5
HGEGTFTSDLSKQMEEEAVRLFIEWLKNGGGGGGGGGGGGGGGAESKYGPPCPPCPAPEAAGGPSVFLFPPKPKDTLMISRTPEVTCVVVDVSQEDPEVQFNWYVDGVEVHNAKTKPREEQFNSTYRVVSVLTVLHQDWLNGKEYKCKVSNKGLPSSIEKTISKAKGQPREPQVYTLPPSQEEMTKNQVSLTCLVKGFYPSDIAVEWESNGQPENNYKTTPPVLDSDGSFFLYSRLTVDKSRWQEGNVFSCSVMHEALHNHYTQKSLSLSLGAPAPAPAPAPAPCP

SEQ ID NO: 118 - protein, 291 aa, Artificial Sequence
  GLP-1 fusion 6
HGEGTFTSDLSKQMEEEAVRLFIEWLKNAPAPAPAPAPAPAPAPAPAPAESKYGPPCPPCPAPEAAGGPSVFLFPPKPKDTLMISRTPEVTCVVVDVSQEDPEVQFNWYVDGVEVHNAKTKPREEQFNSTYRVVSVLTVLHQDWLNGKEYKCKVSNKGLPSSIEKTISKAKGQPREPQVYTLPPSQEEMTKNQVSLTCLVKGFYPSDIAVEWESNGQPENNYKTTPPVLDSDGSFFLYSRLTVDKSRWQEGNVFSCSVMHEALHNHYTQKSLSLSLGAPAPAPAPAPAPCP

SEQ ID NO: 119 - protein, 291 aa, Artificial Sequence
  GLP-1 fusion 7
HGEGTFTSDLSKQMEEEAVRLFIEWLKNAPAPAPAPAPAPAPAPAPAPAPAPAGPPCPPCPAPEAAGGPSVFLFPPKPKDTLMISRTPEVTCVVVDVSQEDPEVQFNWYVDGVEVHNAKTKPREEQFNSTYRVVSVLTVLHQDWLNGKEYKCKVSNKGLPSSIEKTISKAKGQPREPQVYTLPPSQEEMTKNQVSLTCLVKGFYPSDIAVEWESNGQPENNYKTTPPVLDSDGSFFLYSRLTVDKSRWQEGNVFSCSVMHEALHNHYTQKSLSLSLGAPAPAPAPAPAPCP

SEQ ID NO: 120 - protein, 292 aa, Artificial Sequence
  GLP-1 fusion 8
HGEGTFTSDVSSYLEEQAAKEFIAWLVKGGGGGGGAGGGGAGGGGAAESKYGPPCPPCPAPEAAGGPSVFLFPPKPKDTLMISRTPEVTCVVVDVSQEDPEVQFNWYVDGVEVHNAKTKPREEQFNSTYRVVSVLTVLHQDWLNGKEYKCKVSNKGLPSSIEKTISKAKGQPREPQVYTLPPSQEEMTKNQVSLTCLVKGFYPSDIAVEWESNGQPENNYKTTPPVLDSDGSFFLYSRLTVDKSRWQEGNVFSCSVMHEALHNHYTQKSLSLSLGGGGGAGGGGAGGGGACA

SEQ ID NO: 121 - protein, 292 aa, Artificial Sequence
  GLP-1 fusion 9
HGEGTFTSDVSSYLEEQAAKEFIAWLVKGGGGGGGGGGGGGGGGGGAESKYGPPCPPCPAPEAAGGPSVFLFPPKPKDTLMISRTPEVTCVVVDVSQEDPEVQFNWYVDGVEVHNAKTKPREEQFNSTYRVVSVLTVLHQDWLNGKEYKCKVSNKGLPSSIEKTISKAKGQPREPQVYTLPPSQEEMTKNQVSLTCLVKGFYPSDIAVEWESNGQPENNYKTTPPVLDSDGSFFLYSRLTVDKSRWQEGNVFSCSVMHEALHNHYTQKSLSLSLGGGGGAGGGGAGGGGACA

SEQ ID NO: 122 - protein, 297 aa, Artificial Sequence
  GLP-1 fusion 10
HGEGTFTSDVSSYLEEQAAKEFIAWLVKGGGAPAPAPAPAPAPAPAPAPAPAPAPAGPPCPPCPAPEAAGGPSVFLFPPKPKDTLMISRTPEVTCVVVDVSQEDPEVQFNWYVDGVEVHNAKTKPREEQFNSTYRVVSVLTVLHQDWLNGKEYKCKVSNKGLPSSIEKTISKAKGQPREPQVYTLPPSQEEMTKNQVSLTCLVKGFYPSDIAVEWESNGQPENNYKTTPPVLDSDGSFFLYSRLTVDKSRWQEGNVFSCSVMHEALHNHYTQKSLSLSLGGGGGAGGGGAGGGGACA

SEQ ID NO: 123 - protein, 289 aa, Artificial Sequence
  GLP-1 fusion 11
HGEGTFTSDLSKQMEEEAVRLFIEWLKNGGGGAGGGGAGGGGAAESKYGPPCPPCPAPEAAGGPSVFLFPPKPKDTLMISRTPEVTCVVVDVSQEDPEVQFNWYVDGVEVHNAKTKPREEQFNSTYRVVSVLTVLHQDWLNGKEYKCKVSNKGLPSSIEKTISKAKGQPREPQVYTLPPSQEEMTKNQVSLTCLVKGFYPSDIAVEWESNGQPENNYKTTPPVLDSDGSFFLYSRLTVDKSRWQEGNVFSCSVMHEALHNHYTQKSLSLSLGGGGGAGGGGAGGGGACA

SEQ ID NO: 124 - protein, 289 aa, Artificial Sequence
  GLP-1 fusion 12
HGEGTFTSDLSKQMEEEAVRLFIEWLKNGGGGGGGGGGGGGGGAESKYGPPCPPCPAPEAAGGPSVFLFPPKPKDTLMISRTPEVTCVVVDVSQEDPEVQFNWYVDGVEVHNAKTKPREEQFNSTYRVVSVLTVLHQDWLNGKEYKCKVSNKGLPSSIEKTISKAKGQPREPQVYTLPPSQEEMTKNQVSLTCLVKGFYPSDIAVEWESNGQPENNYKTTPPVLDSDGSFFLYSRLTVDKSRWQEGNVFSCSVMHEALHNHYTQKSLSLSLGGGGGAGGGGAGGGGACA

SEQ ID NO: 125 - protein, 294 aa, Artificial Sequence
  GLP-1 fusion 13
HGEGTFTSDLSKQMEEEAVRLFIEWLKNAPAPAPAPAPAPAPAPAPAPAESKYGPPCPPCPAPEAAGGPSVFLFPPKPKDTLMISRTPEVTCVVVDVSQEDPEVQFNWYVDGVEVHNAKTKPREEQFNSTYRVVSVLTVLHQDWLNGKEYKCKVSNKGLPSSIEKTISKAKGQPREPQVYTLPPSQEEMTKNQVSLTCLVKGFYPSDIAVEWESNGQPENNYKTTPPVLDSDGSFFLYSRLTVDKSRWQEGNVFSCSVMHEALHNHYTQKSLSLSLGGGGGAGGGGAGGGGACA

SEQ ID NO: 126 - protein, 294 aa, Artificial Sequence
  GLP-1 fusion 14
HGEGTFTSDLSKQMEEEAVRLFIEWLKNAPAPAPAPAPAPAPAPAPAPAPAPAGPPCPPCPAPEAAGGPSVFLFPPKPKDTLMISRTPEVTCVVVDVSQEDPEVQFNWYVDGVEVHNAKTKPREEQFNSTYRVVSVLTVLHQDWLNGKEYKCKVSNKGLPSSIEKTISKAKGQPREPQVYTLPPSQEEMTKNQVSLTCLVKGFYPSDIAVEWESNGQPENNYKTTPPVLDSDGSFFLYSRLTVDKSRWQEGNVFSCSVMHEALHNHYTQKSLSLSLGGGGGAGGGGAGGGGACA

SEQ ID NO: 127 - protein, 297 aa, Artificial Sequence
  GLP-1 fusion 15
HGEGTFTSDVSSYLEEQAAKEFIAWLVKGGGGGGGAGGGGAGGGGAAESKYGPPCPPCPAPEAAGGPSVFLFPPKPKDTLMISRTPEVTCVVVDVSQEDPEVQFNWYVDGVEVHNAKTKPREEQFNSTYRVVSVLTVLHQDWLNGKEYKCKVSNKGLPSSIEKTISKAKGQPREPQVYTLPPSQEEMTKNQVSLTCLVKGFYPSDIAVEWESNGQPENNYKTTPPVLDSDGSFFLYSRLTVDKSRWQEGNVFSCSVMHEALHNHYTQKSLSLSLGGGGGAYCAKYDGCYGELDFWCQ

SEQ ID NO: 128 - protein, 299 aa, Artificial Sequence
  GLP-1 fusion 16
HGEGTFTSDLSKQMEEEAVRLFIEWLKNAPAPAPAPAPAPAPAPAPAPAPAPAGPPCPPCPAPEAAGGPSVFLFPPKPKDTLMISRTPEVTCVVVDVSQEDPEVQFNWYVDGVEVHNAKTKPREEQFNSTYRVVSVLTVLHQDWLNGKEYKCKVSNKGLPSSIEKTISKAKGQPREPQVYTLPPSQEEMTKNQVSLTCLVKGFYPSDIAVEWESNGQPENNYKTTPPVLDSDGSFFLYSRLTVDKSRWQEGNVFSCSVMHEALHNHYTQKSLSLSLGGGGGAYCAKYDGCYGELDFWCQ

SEQ ID NO: 129 - protein, 297 aa, Artificial Sequence
  GLP-1 fusion 17
HGEGTFTSDVSSYLEEQAAKEFIAWLVKGGGGGGGAGGGGAGGGGAAESKYGPPCPPCPAPEAAGGPSVFLFPPKPKDTLMISRTPEVTCVVVDVSQEDPEVQFNWYVDGVEVHNAKTKPREEQFNSTYRVVSVLTVLHQDWLNGKEYKCKVSNKGLPSSIEKTISKAKGQPREPQVYTLPPSQEEMTKNQVSLTCLVKGFYPSDIAVEWESNGQPENNYKTTPPVLDSDGSFFLYSRLTVDKSRWQEGNVFSCSVMHEALHNHYTQKSLSLSLGGGGGAYSAKYDGCYGELDFWGQ

SEQ ID NO: 130 - protein, 299 aa, Artificial Sequence
  GLP-1 fusion 18
HGEGTFTSDLSKQMEEEAVRLFIEWLKNAPAPAPAPAPAPAPAPAPAPAPAPAGPPCPPCPAPEAAGGPSVFLFPPKPKDTLMISRTPEVTCVVVDVSQEDPEVQFNWYVDGVEVHNAKTKPREEQFNSTYRVVSVLTVLHQDWLNGKEYKCKVSNKGLPSSIEKTISKAKGQPREPQVYTLPPSQEEMTKNQVSLTCLVKGFYPSDIAVEWESNGQPENNYKTTPPVLDSDGSFFLYSRLTVDKSRWQEGNVFSCSVMHEALHNHYTQKSLSLSLGGGGGAYSAKYDGCYGELDFWGQ

SEQ ID NO: 131 - protein, 290 aa, Artificial Sequence
  GLP-1 fusion 19
HGEGTFTSDVSSYLEEQAAKEFIAWLVKGGGGGGGAGGGGAGGGGAAESKYGPPCPPCPAPEAAGGPSVFLFPPKPKDTLMISRTPEVTCVVVDVSQEDPEVQFNWYVDGVEVHNAKTKPREEQFNSTYRVVSVLTVLHQDWLNGKEYKCKVSNKGLPSSIEKTISKAKGQPREPQVYTLPPSQEEMTKNQVSLTCLVKGFYPSDIAVEWESNGQPENNYKTTPPVLDSDGSFFLYSRLTVDKSRWQEGNVFSCSVMHEALHNHYTQKSLSLSLGGGGAPAPAPEEEPCA

SEQ ID NO: 132 - protein, 290 aa, Artificial Sequence
  GLP-1 fusion 20
HGEGTFTSDVSSYLEEQAAKEFIAWLVKGGGGGGGGGGGGGGGGGGAESKYGPPCPPCPAPEAAGGPSVFLFPPKPKDTLMISRTPEVTCVVVDVSQEDPEVQFNWYVDGVEVHNAKTKPREEQFNSTYRVVSVLTVLHQDWLNGKEYKCKVSNKGLPSSIEKTISKAKGQPREPQVYTLPPSQEEMTKNQVSLTCLVKGFYPSDIAVEWESNGQPENNYKTTPPVLDSDGSFFLYSRLTVDKSRWQEGNVFSCSVMHEALHNHYTQKSLSLSLGGGGAPAPAPEEEPCA

SEQ ID NO: 133 - protein, 287 aa, Artificial Sequence
  GLP-1 fusion 21
HGEGTFTSDLSKQMEEEAVRLFIEWLKNGGGGAGGGGAGGGGAAESKYGPPCPPCPAPEAAGGPSVFLFPPKPKDTLMISRTPEVTCVVVDVSQEDPEVQFNWYVDGVEVHNAKTKPREEQFNSTYRVVSVLTVLHQDWLNGKEYKCKVSNKGLPSSIEKTISKAKGQPREPQVYTLPPSQEEMTKNQVSLTCLVKGFYPSDIAVEWESNGQPENNYKTTPPVLDSDGSFFLYSRLTVDKSRWQEGNVFSCSVMHEALHNHYTQKSLSLSLGGGGAPAPAPEEEPCA

SEQ ID NO: 134 - protein, 298 aa, Artificial Sequence
  GLP-1 fusion 22
HGEGTFTSDLSKQMEEEAVRLFIEWLKNGGPSSGAPPPSGGGGAGGGGAGGGGAAESKYGPPCPPCPAPEAAGGPSVFLFPPKPKDTLMISRTPEVTCVVVDVSQEDPEVQFNWYVDGVEVHNAKTKPREEQFNSTYRVVSVLTVLHQDWLNGKEYKCKVSNKGLPSSIEKTISKAKGQPREPQVYTLPPSQEEMTKNQVSLTCLVKGFYPSDIAVEWESNGQPENNYKTTPPVLDSDGSFFLYSRLTVDKSRWQEGNVFSCSVMHEALHNHYTQKSLSLSLGGGGAPAPAPEEEPCA

SEQ ID NO: 135 - protein, 298 aa, Artificial Sequence
  GLP-1 fusion 23
HGEGTFTSDLSKQMEEEAVRLFIEWLKNGGPSSGAPPPSGGGGGGGGGGGGGGGAESKYGPPCPPCPAPEAAGGPSVFLFPPKPKDTLMISRTPEVTCVVVDVSQEDPEVQFNWYVDGVEVHNAKTKPREEQFNSTYRVVSVLTVLHQDWLNGKEYKCKVSNKGLPSSIEKTISKAKGQPREPQVYTLPPSQEEMTKNQVSLTCLVKGFYPSDIAVEWESNGQPENNYKTTPPVLDSDGSFFLYSRLTVDKSRWQEGNVFSCSVMHEALHNHYTQKSLSLSLGGGGAPAPAPEEEPCA

SEQ ID NO: 136 - protein, 292 aa, Artificial Sequence
  GLP-1 fusion 24
HGEGTFTSDVSSYLEEQAAKEFIAWLVKGGGGGGGAGGGGAGGGGAAESKYGPPCPPCPAPEAAGGPSVFLFPPKPKDTLMISRTPEVTCVVVDVSQEDPEVQFNWYVDGVEVHNAKTKPREEQFNSTYRVVSVLTVLHQDWLNGKEYKCKVSNKGLPSSIEKTISKAKGQPREPQVYTLPPSQEEMTKNQVSLTCLVKGFYPSDIAVEWESNGQPENNYKTTPPVLDSDGSFFLYSRLTVDKSRWQEGNVFSCSVMHEALHNHYTQKSLSLSLGAPAPAPAPAPAPCPEEP

SEQ ID NO: 137 - protein, 292 aa, Artificial Sequence
  GLP-1 fusion 25
HGEGTFTSDVSSYLEEQAAKEFIAWLVKGGGGGGGGGGGGGGGGGGAESKYGPPCPPCPAPEAAGGPSVFLFPPKPKDTLMISRTPEVTCVVVDVSQEDPEVQFNWYVDGVEVHNAKTKPREEQFNSTYRVVSVLTVLHQDWLNGKEYKCKVSNKGLPSSIEKTISKAKGQPREPQVYTLPPSQEEMTKNQVSLTCLVKGFYPSDIAVEWESNGQPENNYKTTPPVLDSDGSFFLYSRLTVDKSRWQEGNVFSCSVMHEALHNHYTQKSLSLSLGAPAPAPAPAPAPCPEEP

SEQ ID NO: 138 - protein, 297 aa, Artificial Sequence
  GLP-1 fusion 26
HGEGTFTSDVSSYLEEQAAKEFIAWLVKGGGAPAPAPAPAPAPAPAPAPAPAESKYGPPCPPCPAPEAAGGPSVFLFPPKPKDTLMISRTPEVTCVVVDVSQEDPEVQFNWYVDGVEVHNAKTKPREEQFNSTYRVVSVLTVLHQDWLNGKEYKCKVSNKGLPSSIEKTISKAKGQPREPQVYTLPPSQEEMTKNQVSLTCLVKGFYPSDIAVEWESNGQPENNYKTTPPVLDSDGSFFLYSRLTVDKSRWQEGNVFSCSVMHEALHNHYTQKSLSLSLGAPAPAPAPAPAPCPEEP

SEQ ID NO: 139 - protein, 297 aa, Artificial Sequence
  GLP-1 fusion 27
HGEGTFTSDVSSYLEEQAAKEFIAWLVKGGGAPAPAPAPAPAPAPAPAPAPAPAPAGPPCPPCPAPEAAGGPSVFLFPPKPKDTLMISRTPEVTCVVVDVSQEDPEVQFNWYVDGVEVHNAKTKPREEQFNSTYRVVSVLTVLHQDWLNGKEYKCKVSNKGLPSSIEKTISKAKGQPREPQVYTLPPSQEEMTKNQVSLTCLVKGFYPSDIAVEWESNGQPENNYKTTPPVLDSDGSFFLYSRLTVDKSRWQEGNVFSCSVMHEALHNHYTQKSLSLSLGAPAPAPAPAPAPCPEEP

SEQ ID NO: 140 - protein, 289 aa, Artificial Sequence
  GLP-1 fusion 28
HGEGTFTSDLSKQMEEEAVRLFIEWLKNGGGGAGGGGAGGGGAAESKYGPPCPPCPAPEAAGGPSVFLFPPKPKDTLMISRTPEVTCVVVDVSQEDPEVQFNWYVDGVEVHNAKTKPREEQFNSTYRVVSVLTVLHQDWLNGKEYKCKVSNKGLPSSIEKTISKAKGQPREPQVYTLPPSQEEMTKNQVSLTCLVKGFYPSDIAVEWESNGQPENNYKTTPPVLDSDGSFFLYSRLTVDKSRWQEGNVFSCSVMHEALHNHYTQKSLSLSLGAPAPAPAPAPAPCPEEP

SEQ ID NO: 141 - protein, 289 aa, Artificial Sequence
  GLP-1 fusion 29
HGEGTFTSDLSKQMEEEAVRLFIEWLKNGGGGGGGGGGGGGGGAESKYGPPCPPCPAPEAAGGPSVFLFPPKPKDTLMISRTPEVTCVVVDVSQEDPEVQFNWYVDGVEVHNAKTKPREEQFNSTYRVVSVLTVLHQDWLNGKEYKCKVSNKGLPSSIEKTISKAKGQPREPQVYTLPPSQEEMTKNQVSLTCLVKGFYPSDIAVEWESNGQPENNYKTTPPVLDSDGSFFLYSRLTVDKSRWQEGNVFSCSVMHEALHNHYTQKSLSLSLGAPAPAPAPAPAPCPEEP

SEQ ID NO: 142 - protein, 294 aa, Artificial Sequence
  GLP-1 fusion 30
HGEGTFTSDLSKQMEEEAVRLFIEWLKNAPAPAPAPAPAPAPAPAPAPAESKYGPPCPPCPAPEAAGGPSVFLFPPKPKDTLMISRTPEVTCVVVDVSQEDPEVQFNWYVDGVEVHNAKTKPREEQFNSTYRVVSVLTVLHQDWLNGKEYKCKVSNKGLPSSIEKTISKAKGQPREPQVYTLPPSQEEMTKNQVSLTCLVKGFYPSDIAVEWESNGQPENNYKTTPPVLDSDGSFFLYSRLTVDKSRWQEGNVFSCSVMHEALHNHYTQKSLSLSLGAPAPAPAPAPAPCPEEP

SEQ ID NO: 143 - protein, 294 aa, Artificial Sequence
  GLP-1 fusion 31
HGEGTFTSDLSKQMEEEAVRLFIEWLKNAPAPAPAPAPAPAPAPAPAPAPAPAGPPCPPCPAPEAAGGPSVFLFPPKPKDTLMISRTPEVTCVVVDVSQEDPEVQFNWYVDGVEVHNAKTKPREEQFNSTYRVVSVLTVLHQDWLNGKEYKCKVSNKGLPSSIEKTISKAKGQPREPQVYTLPPSQEEMTKNQVSLTCLVKGFYPSDIAVEWESNGQPENNYKTTPPVLDSDGSFFLYSRLTVDKSRWQEGNVFSCSVMHEALHNHYTQKSLSLSLGAPAPAPAPAPAPCPEEP

SEQ ID NO: 144 - protein, 280 aa, Artificial Sequence
  GLP-1 fusion 32
HSEGTFTSDVSSYLEGQAAKEFIEWLVKGRASGGGGSGGGGSCPPCPAPEAAGGPSVFLFPPKPKDTLMISRTPEVTCVVVDVSQEDPEVQFNWYVDGVEVHNAKTKPREEQFNSTYRVVSVLTVLHQDWLNGKEYKCKVSNKGLPSSIEKTISKAKGQPREPQVYTLPPSQEEMTKNQVSLTCLVKGFYPSDIAVEWESNGQPENNYKTTPPVLDSDGSFFLYSRLTVDKSRWQEGNVFSCSVMHEALHNHYTQKSLSLSLGKASGSAPAPAPEEEPCA

SEQ ID NO: 145 - protein, 282 aa, Artificial Sequence
  GLP-1 fusion 33
HSEGTFTSDVSSYLEGQAAKEFIEWLVKGRASAPAPAPAPAPGSCPPCPAPEAAGGPSVFLFPPKPKDTLMISRTPEVTCVVVDVSQEDPEVQFNWYVDGVEVHNAKTKPREEQFNSTYRVVSVLTVLHQDWLNGKEYKCKVSNKGLPSSIEKTISKAKGQPREPQVYTLPPSQEEMTKNQVSLTCLVKGFYPSDIAVEWESNGQPENNYKTTPPVLDSDGSFFLYSRLTVDKSRWQEGNVFSCSVMHEALHNHYTQKSLSLSLGKASGSAPAPAPEEEPCA

SEQ ID NO: 146 - protein, 289 aa, Artificial Sequence
  GLP-1 fusion 34
HGEGTFTSDLSKQMEEEAVRLFIEWLKNGGPSSGAPPPSASGGGGSGGGGSCPPCPAPEAAGGPSVFLFPPKPKDTLMISRTPEVTCVVVDVSQEDPEVQFNWYVDGVEVHNAKTKPREEQFNSTYRVVSVLTVLHQDWLNGKEYKCKVSNKGLPSSIEKTISKAKGQPREPQVYTLPPSQEEMTKNQVSLTCLVKGFYPSDIAVEWESNGQPENNYKTTPPVLDSDGSFFLYSRLTVDKSRWQEGNVFSCSVMHEALHNHYTQKSLSLSLGKASGSAPAPAPEEEPCA

SEQ ID NO: 147 - protein, 291 aa, Artificial Sequence
  GLP-1 fusion 35
HGEGTFTSDLSKQMEEEAVRLFIEWLKNGGPSSGAPPPSASAPAPAPAPAPGSCPPCPAPEAAGGPSVFLFPPKPKDTLMISRTPEVTCVVVDVSQEDPEVQFNWYVDGVEVHNAKTKPREEQFNSTYRVVSVLTVLHQDWLNGKEYKCKVSNKGLPSSIEKTISKAKGQPREPQVYTLPPSQEEMTKNQVSLTCLVKGFYPSDIAVEWESNGQPENNYKTTPPVLDSDGSFFLYSRLTVDKSRWQEGNVFSCSVMHEALHNHYTQKSLSLSLGKASGSAPAPAPEEEPCA

SEQ ID NO: 148 - protein, 283 aa, Artificial Sequence
  GLP-1 fusion 36
HSEGTFTSDVSSYLEGQAAKEFIEWLVKGRASGGGGSGGGGSGPPCPPCPAPEAAGGPSVFLFPPKPKDTLMISRTPEVTCVVVDVSQEDPEVQFNWYVDGVEVHNAKTKPREEQFNSTYRVVSVLTVLHQDWLNGKEYKCKVSNKGLPSSIEKTISKAKGQPREPQVYTLPPSQEEMTKNQVSLTCLVKGFYPSDIAVEWESNGQPENNYKTTPPVLDSDGSFFLYSRLTVDKSRWQEGNVFSCSVMHEALHNHYTQKSLSLSLGKASGSAPAPAPEEEPCA

SEQ ID NO: 149 - protein, 292 aa, Artificial Sequence
  GLP-1 fusion 37
HGEGTFTSDLSKQMEEEAVRLFIEWLKNGGPSSGAPPPSASGGGGSGGGGSGPPCPPCPAPEAAGGPSVFLFPPKPKDTLMISRTPEVTCVVVDVSQEDPEVQFNWYVDGVEVHNAKTKPREEQFNSTYRVVSVLTVLHQDWLNGKEYKCKVSNKGLPSSIEKTISKAKGQPREPQVYTLPPSQEEMTKNQVSLTCLVKGFYPSDIAVEWESNGQPENNYKTTPPVLDSDGSFFLYSRLTVDKSRWQEGNVFSCSVMHEALHNHYTQKSLSLSLGKASGSAPAPAPEEEPCA

SEQ ID NO: 150 - protein, 290 aa, Artificial Sequence
  GLP-1 fusion 38
HSEGTFTSDVSSYLEGQAAKEFIEWLVKGRASGGGGSGGGGSGGGGSGGGGSCPPCPAPEAAGGPSVFLFPPKPKDTLMISRTPEVTCVVVDVSQEDPEVQFNWYVDGVEVHNAKTKPREEQFNSTYRVVSVLTVLHQDWLNGKEYKCKVSNKGLPSSIEKTISKAKGQPREPQVYTLPPSQEEMTKNQVSLTCLVKGFYPSDIAVEWESNGQPENNYKTTPPVLDSDGSFFLYSRLTVDKSRWQEGNVFSCSVMHEALHNHYTQKSLSLSLGKASGSAPAPAPEEEPCA

SEQ ID NO: 151 - protein, 292 aa, Artificial Sequence
  GLP-1 fusion 39
HSEGTFTSDVSSYLEGQAAKEFIEWLVKGRASAPAPAPAPAPAPAPAPAPAPGSCPPCPAPEAAGGPSVFLFPPKPKDTLMISRTPEVTCVVVDVSQEDPEVQFNWYVDGVEVHNAKTKPREEQFNSTYRVVSVLTVLHQDWLNGKEYKCKVSNKGLPSSIEKTISKAKGQPREPQVYTLPPSQEEMTKNQVSLTCLVKGFYPSDIAVEWESNGQPENNYKTTPPVLDSDGSFFLYSRLTVDKSRWQEGNVFSCSVMHEALHNHYTQKSLSLSLGKASGSAPAPAPEEEPCA

SEQ ID NO: 152 - protein, 281 aa, Artificial Sequence
  GLP-1 fusion 40
HGEGTFTSDVSSYLEEQAAKEFIAWLVKGGGASGGGGSGGGGSCPPCPAPEAAGGPSVFLFPPKPKDTLMISRTPEVTCVVVDVSQEDPEVQFNWYVDGVEVHNAKTKPREEQFNSTYRVVSVLTVLHQDWLNGKEYKCKVSNKGLPSSIEKTISKAKGQPREPQVYTLPPSQEEMTKNQVSLTCLVKGFYPSDIAVEWESNGQPENNYKTTPPVLDSDGSFFLYSRLTVDKSRWQEGNVFSCSVMHEALHNHYTQKSLSLSLGKASGSAPAPAPEEEPCA

SEQ ID NO: 153 - protein, 291 aa, Artificial Sequence
  GLP-1 fusion 41
HGEGTFTSDVSSYLEEQAAKEFIAWLVKGGGASGGGGSGGGGSGGGGSGGGGSCPPCPAPEAAGGPSVFLFPPKPKDTLMISRTPEVTCVVVDVSQEDPEVQFNWYVDGVEVHNAKTKPREEQFNSTYRVVSVLTVLHQDWLNGKEYKCKVSNKGLPSSIEKTISKAKGQPREPQVYTLPPSQEEMTKNQVSLTCLVKGFYPSDIAVEWESNGQPENNYKTTPPVLDSDGSFFLYSRLTVDKSRWQEGNVFSCSVMHEALHNHYTQKSLSLSLGKASGSAPAPAPEEEPCA

SEQ ID NO: 154 - protein, 289 aa, Artificial Sequence
  GLP-1 fusion 42
HGEGTFTSDLSKQMEEEAVRLFIEWLKNGGPSSGAPPPSASGGGGSGGGGSCPPCPAPEAAGGPSVFLFPPKPKDTLMISRTPEVTCVVVDVSQEDPEVQFNWYVDGVEVHNAKTKPREEQFNSTYRVVSVLTVLHQDWLNGKEYKCKVSNKGLPSSIEKTISKAKGQPREPQVYTLPPSQEEMTKNQVSLTCLVKGFYPSDIAVEWESNGQPENNYKTTPPVLDSDGSFFLYSRLTVDKSRWQEGNVFSCSVMHEALHNHYTQKSLSLSLGKASGSAPAPEPEPEPCA

SEQ ID NO: 155 - protein, 291 aa, Artificial Sequence
  GLP-1 fusion 43
HGEGTFTSDLSKQMEEEAVRLFIEWLKNGGPSSGAPPPSASAPAPAPAPAPGSCPPCPAPEAAGGPSVFLFPPKPKDTLMISRTPEVTCVVVDVSQEDPEVQFNWYVDGVEVHNAKTKPREEQFNSTYRVVSVLTVLHQDWLNGKEYKCKVSNKGLPSSIEKTISKAKGQPREPQVYTLPPSQEEMTKNQVSLTCLVKGFYPSDIAVEWESNGQPENNYKTTPPVLDSDGSFFLYSRLTVDKSRWQEGNVFSCSVMHEALHNHYTQKSLSLSLGKASGSAPAPEPEPEPCA

SEQ ID NO: 156 - protein, 281 aa, Artificial Sequence
  GLP-1 fusion 44
HGEGTFTSDVSSYLEEQAAKEFIAWLVKGGGASGGGGSGGGGSCPPCPAPEAAGGPSVFLFPPKPKDTLMISRTPEVTCVVVDVSQEDPEVQFNWYVDGVEVHNAKTKPREEQFNSTYRVVSVLTVLHQDWLNGKEYKCKVSNKGLPSSIEKTISKAKGQPREPQVYTLPPSQEEMTKNQVSLTCLVKGFYPSDIAVEWESNGQPENNYKTTPPVLDSDGSFFLYSRLTVDKSRWQEGNVFSCSVMHEALHNHYTQKSLSLSLGKASGSAPAPEPEPEPCA

SEQ ID NO: 157 - protein, 289 aa, Artificial Sequence
  GLP-1 fusion 45
HGEGTFTSDLSKQMEEEAVRLFIEWLKNGGPSSGAPPPSASGGGGSGGGGSCPPCPAPEAAGGPSVFLFPPKPKDTLMISRTPEVTCVVVDVSQEDPEVQFNWYVDGVEVHNAKTKPREEQFNSTYRVVSVLTVLHQDWLNGKEYKCKVSNKGLPSSIEKTISKAKGQPREPQVYTLPPSQEEMTKNQVSLTCLVKGFYPSDIAVEWESNGQPENNYKTTPPVLDSDGSFFLYSRLTVDKSRWQEGNVFSCSVMHEALHNHYTQKSLSLSLGKASGSAPAPAPAPCEEE

SEQ ID NO: 158 - protein, 291 aa, Artificial Sequence
  GLP-1 fusion 46
HGEGTFTSDLSKQMEEEAVRLFIEWLKNGGPSSGAPPPSASAPAPAPAPAPGSCPPCPAPEAAGGPSVFLFPPKPKDTLMISRTPEVTCVVVDVSQEDPEVQFNWYVDGVEVHNAKTKPREEQFNSTYRVVSVLTVLHQDWLNGKEYKCKVSNKGLPSSIEKTISKAKGQPREPQVYTLPPSQEEMTKNQVSLTCLVKGFYPSDIAVEWESNGQPENNYKTTPPVLDSDGSFFLYSRLTVDKSRWQEGNVFSCSVMHEALHNHYTQKSLSLSLGKASGSAPAPAPAPCEEE

SEQ ID NO: 159 - protein, 292 aa, Artificial Sequence
  GLP-1 fusion 47
HGEGTFTSDLSKQMEEEAVRLFIEWLKNGGPSSGAPPPSASGGGGSGGGGSGPPCPPCPAPEAAGGPSVFLFPPKPKDTLMISRTPEVTCVVVDVSQEDPEVQFNWYVDGVEVHNAKTKPREEQFNSTYRVVSVLTVLHQDWLNGKEYKCKVSNKGLPSSIEKTISKAKGQPREPQVYTLPPSQEEMTKNQVSLTCLVKGFYPSDIAVEWESNGQPENNYKTTPPVLDSDGSFFLYSRLTVDKSRWQEGNVFSCSVMHEALHNHYTQKSLSLSLGKASGSAPAPAPAPCEEE

SEQ ID NO: 160 - protein, 281 aa, Artificial Sequence
  GLP-1 fusion 48
HGEGTFTSDVSSYLEEQAAKEFIAWLVKGGGASGGGGSGGGGSCPPCPAPEAAGGPSVFLFPPKPKDTLMISRTPEVTCVVVDVSQEDPEVQFNWYVDGVEVHNAKTKPREEQFNSTYRVVSVLTVLHQDWLNGKEYKCKVSNKGLPSSIEKTISKAKGQPREPQVYTLPPSQEEMTKNQVSLTCLVKGFYPSDIAVEWESNGQPENNYKTTPPVLDSDGSFFLYSRLTVDKSRWQEGNVFSCSVMHEALHNHYTQKSLSLSLGKASGSAPAPAPAPCEEE

SEQ ID NO: 161 - protein, 290 aa, Artificial Sequence
  GLP-1 fusion 49
HGEGTFTSDLSKQMEEEAVRLFIEWLKNGGPSSGAPPPSASGGGGSGGGGSCPPCPAPEAAGGPSVFLFPPKPKDTLMISRTPEVTCVVVDVSQEDPEVQFNWYVDGVEVHNAKTKPREEQFNSTYRVVSVLTVLHQDWLNGKEYKCKVSNKGLPSSIEKTISKAKGQPREPQVYTLPPSQEEMTKNQVSLTCLVKGFYPSDIAVEWESNGQPENNYKTTPPVLDSDGSFFLYSRLTVDKSRWQEGNVFSCSVMHEALHNHYTQKSLSLSLGKASGSAPAPAPAPCPEEP

SEQ ID NO: 162 - protein, 292 aa, Artificial Sequence
  GLP-1 fusion 50
HGEGTFTSDLSKQMEEEAVRLFIEWLKNGGPSSGAPPPSASAPAPAPAPAPGSCPPCPAPEAAGGPSVFLFPPKPKDTLMISRTPEVTCVVVDVSQEDPEVQFNWYVDGVEVHNAKTKPREEQFNSTYRVVSVLTVLHQDWLNGKEYKCKVSNKGLPSSIEKTISKAKGQPREPQVYTLPPSQEEMTKNQVSLTCLVKGFYPSDIAVEWESNGQPENNYKTTPPVLDSDGSFFLYSRLTVDKSRWQEGNVFSCSVMHEALHNHYTQKSLSLSLGKASGSAPAPAPAPCPEEP

SEQ ID NO: 163 - protein, 293 aa, Artificial Sequence
  GLP-1 fusion 51
HGEGTFTSDLSKQMEEEAVRLFIEWLKNGGPSSGAPPPSASGGGGSGGGGSGPPCPPCPAPEAAGGPSVFLFPPKPKDTLMISRTPEVTCVVVDVSQEDPEVQFNWYVDGVEVHNAKTKPREEQFNSTYRVVSVLTVLHQDWLNGKEYKCKVSNKGLPSSIEKTISKAKGQPREPQVYTLPPSQEEMTKNQVSLTCLVKGFYPSDIAVEWESNGQPENNYKTTPPVLDSDGSFFLYSRLTVDKSRWQEGNVFSCSVMHEALHNHYTQKSLSLSLGKASGSAPAPAPAPCPEEP

SEQ ID NO: 164 - protein, 282 aa, Artificial Sequence
  GLP-1 fusion 52
HGEGTFTSDVSSYLEEQAAKEFIAWLVKGGGASGGGGSGGGGSCPPCPAPEAAGGPSVFLFPPKPKDTLMISRTPEVTCVVVDVSQEDPEVQFNWYVDGVEVHNAKTKPREEQFNSTYRVVSVLTVLHQDWLNGKEYKCKVSNKGLPSSIEKTISKAKGQPREPQVYTLPPSQEEMTKNQVSLTCLVKGFYPSDIAVEWESNGQPENNYKTTPPVLDSDGSFFLYSRLTVDKSRWQEGNVFSCSVMHEALHNHYTQKSLSLSLGKASGSAPAPAPAPCPEEP

SEQ ID NO: 165 - protein, 283 aa, Artificial Sequence
  GLP-1 fusion 53
HGEGTFTSDVSSYLEEQAAKEFIAWLVKGGGASAPAPAPAPAPGSCPPCPAPEAAGGPSVFLFPPKPKDTLMISRTPEVTCVVVDVSQEDPEVQFNWYVDGVEVHNAKTKPREEQFNSTYRVVSVLTVLHQDWLNGKEYKCKVSNKGLPSSIEKTISKAKGQPREPQVYTLPPSQEEMTKNQVSLTCLVKGFYPSDIAVEWESNGQPENNYKTTPPVLDSDGSFFLYSRLTVDKSRWQEGNVFSCSVMHEALHNHYTQKSLSLSLGKASGSAPAPAPEEEPCA

SEQ ID NO: 166 - protein, 293 aa, Artificial Sequence
  GLP-1 fusion 54
HGEGTFTSDVSSYLEEQAAKEFIAWLVKGGGASAPAPAPAPAPAPAPAPAPAPGSCPPCPAPEAAGGPSVFLFPPKPKDTLMISRTPEVTCVVVDVSQEDPEVQFNWYVDGVEVHNAKTKPREEQFNSTYRVVSVLTVLHQDWLNGKEYKCKVSNKGLPSSIEKTISKAKGQPREPQVYTLPPSQEEMTKNQVSLTCLVKGFYPSDIAVEWESNGQPENNYKTTPPVLDSDGSFFLYSRLTVDKSRWQEGNVFSCSVMHEALHNHYTQKSLSLSLGKASGSAPAPAPEEEPCA

SEQ ID NO: 167 - protein, 277 aa, Artificial Sequence
  GLP-1 fusion 55
HGEGTFTSDLSKQMEEEAVRLFIEWLKNGGPSSGAPPPSCPPCPAPEAAGGPSVFLFPPKPKDTLMISRTPEVTCVVVDVSQEDPEVQFNWYVDGVEVHNAKTKPREEQFNSTYRVVSVLTVLHQDWLNGKEYKCKVSNKGLPSSIEKTISKAKGQPREPQVYTLPPSQEEMTKNQVSLTCLVKGFYPSDIAVEWESNGQPENNYKTTPPVLDSDGSFFLYSRLTVDKSRWQEGNVFSCSVMHEALHNHYTQKSLSLSLGKASGSAPAPAPEEEPCA

SEQ ID NO: 168 - protein, 283 aa, Artificial Sequence
  GLP-1 fusion 56
HGEGTFTSDLSKQMEEEAVRLFIEWLKNGGPSSGAPPPSGGGGGGCPPCPAPEAAGGPSVFLFPPKPKDTLMISRTPEVTCVVVDVSQEDPEVQFNWYVDGVEVHNAKTKPREEQFNSTYRVVSVLTVLHQDWLNGKEYKCKVSNKGLPSSIEKTISKAKGQPREPQVYTLPPSQEEMTKNQVSLTCLVKGFYPSDIAVEWESNGQPENNYKTTPPVLDSDGSFFLYSRLTVDKSRWQEGNVFSCSVMHEALHNHYTQKSLSLSLGKASGSAPAPAPEEEPCA

SEQ ID NO: 169 - protein, 283 aa, Artificial Sequence
  GLP-1 fusion 57
HGEGTFTSDLSKQMEEEAVRLFIEWLKNGGPSSGAPPPSAPAPAPCPPCPAPEAAGGPSVFLFPPKPKDTLMISRTPEVTCVVVDVSQEDPEVQFNWYVDGVEVHNAKTKPREEQFNSTYRVVSVLTVLHQDWLNGKEYKCKVSNKGLPSSIEKTISKAKGQPREPQVYTLPPSQEEMTKNQVSLTCLVKGFYPSDIAVEWESNGQPENNYKTTPPVLDSDGSFFLYSRLTVDKSRWQEGNVFSCSVMHEALHNHYTQKSLSLSLGKASGSAPAPAPEEEPCA

SEQ ID NO: 170 - protein, 282 aa, Artificial Sequence
  GLP-1 fusion 58
HGEGTFTSDLSKQMEEEAVRLFIEWLKNGGPSSGAPPPSASGGGGSGGGGSCPPCPAPEAAGGPSVFLFPPKPKDTLMISRTPEVTCVVVDVSQEDPEVQFNWYVDGVEVHNAKTKPREEQFNSTYRVVSVLTVLHQDWLNGKEYKCKVSNKGLPSSIEKTISKAKGQPREPQVYTLPPSQEEMTKNQVSLTCLVKGFYPSDIAVEWESNGQPENNYKTTPPVLDSDGSFFLYSRLTVDKSRWQEGNVFSCSVMHEALHNHYTQKSLSLSLGKAPAPEEPCA

SEQ ID NO: 171 - protein, 281 aa, Artificial Sequence
  GLP-1 fusion 59
HGEGTFTSDLSKQMEEEAVRLFIEWLKNGGPSSGAPPPSASGGGGSGGGGSCPPCPAPEAAGGPSVFLFPPKPKDTLMISRTPEVTCVVVDVSQEDPEVQFNWYVDGVEVHNAKTKPREEQFNSTYRVVSVLTVLHQDWLNGKEYKCKVSNKGLPSSIEKTISKAKGQPREPQVYTLPPSQEEMTKNQVSLTCLVKGFYPSDIAVEWESNGQPENNYKTTPPVLDSDGSFFLYSRLTVDKSRWQEGNVFSCSVMHEALHNHYTQKSLSLSLGKAAAEEPCA

SEQ ID NO: 172 - protein, 287 aa, Artificial Sequence
  GLP-1 fusion 60
HGEGTFTSDLSKQMEEEAVRLFIEWLKNGGPSSGAPPPSASGGGGSGGGGSCPPCPAPEAAGGPSVFLFPPKPKDTLMISRTPEVTCVVVDVSQEDPEVQFNWYVDGVEVHNAKTKPREEQFNSTYRVVSVLTVLHQDWLNGKEYKCKVSNKGLPSSIEKTISKAKGQPREPQVYTLPPSQEEMTKNQVSLTCLVKGFYPSDIAVEWESNGQPENNYKTTPPVLDSDGSFFLYSRLTVDKSRWQEGNVFSCSVMHEALHNHYTQKSLSLSLGKAPAPAPAPCAPRRR

SEQ ID NO: 173 - protein, 281 aa, Artificial Sequence
  GLP-1 fusion 61
HGEGTFTSDLSKQMEEEAVRLFIEWLKNGGPSSGAPPPSASGGGGSGGGGSCPPCPAPEAAGGPSVFLFPPKPKDTLMISRTPEVTCVVVDVSQEDPEVQFNWYVDGVEVHNAKTKPREEQFNSTYRVVSVLTVLHQDWLNGKEYKCKVSNKGLPSSIEKTISKAKGQPREPQVYTLPPSQEEMTKNQVSLTCLVKGFYPSDIAVEWESNGQPENNYKTTPPVLDSDGSFFLYSRLTVDKSRWQEGNVFSCSVMHEALHNHYTQKSLSLSLGKAAACPEEE

SEQ ID NO: 174 - protein, 289 aa, Artificial Sequence
  GLP-1 fusion 62
HGEGTFTSDLSKQMEEEAVRLFIEWLKNGGPSSGAPPPSASGGGGSGGGGSCPPCPAPEAAGGPSVFLFPPKPKDTLMISRTPEVTCVVVDVSQEDPEVQFNWYVDGVEVHNAKTKPREEQFNSTYRVVSVLTVLHQDWLNGKEYKCKVSNKGLPSSIEKTISKAKGQPREPQVYTLPPSQEEMTKNQVSLTCLVKGFYPSDIAVEWESNGQPENNYKTTPPVLDSDGSFFLYSRLTVDKSRWQEGNVFSCSVMHEALHNHYTQKSLSLSLGKASGSGGGGSGGGGSCA

SEQ ID NO: 175 - protein, 297 aa, Artificial Sequence
  GLP-1 fusion 63
HGEGTFTSDVSSYLEEQAAKEFIAWLVKGGGAPAPAPAPAPAPAPAPAPAPAESKYGPPCPPCPAPEAAGGPSVFLFPPKPKDTLMISRTPEVTCVVVDVSQEDPEVQFNWYVDGVEVHNAKTKPREEQFNSTYRVVSVLTVLHQDWLNGKEYKCKVSNKGLPSSIEKTISKAKGQPREPQVYTLPPSQEEMTKNQVSLTCLVKGFYPSDIAVEWESNGQPENNYKTTPPVLDSDGSFFLYSRLTVDKSRWQEGNVFSCSVMHEALHNHYTQKSLSLSLGKASGSAPAPAPEEEPCA

SEQ ID NO: 176 - protein, 305 aa, Artificial Sequence
  GLP-1 fusion 64
HGEGTFTSDLSKQMEEEAVRLFIEWLKNGGPSSGAPPPSAPAPAPAPAPAPAPAPAPAPAESKYGPPCPPCPAPEAAGGPSVFLFPPKPKDTLMISRTPEVTCVVVDVSQEDPEVQFNWYVDGVEVHNAKTKPREEQFNSTYRVVSVLTVLHQDWLNGKEYKCKVSNKGLPSSIEKTISKAKGQPREPQVYTLPPSQEEMTKNQVSLTCLVKGFYPSDIAVEWESNGQPENNYKTTPPVLDSDGSFFLYSRLTVDKSRWQEGNVFSCSVMHEALHNHYTQKSLSLSLGKASGSAPAPAPEEEPCA

SEQ ID NO: 177 - protein, 294 aa, Artificial Sequence
  GLP-1 fusion 65
HGEGTFTSDLSKQMEEEAVRLFIEWLKNAPAPAPAPAPAPAPAPAPAPAESKYGPPCPPCPAPEAAGGPSVFLFPPKPKDTLMISRTPEVTCVVVDVSQEDPEVQFNWYVDGVEVHNAKTKPREEQFNSTYRVVSVLTVLHQDWLNGKEYKCKVSNKGLPSSIEKTISKAKGQPREPQVYTLPPSQEEMTKNQVSLTCLVKGFYPSDIAVEWESNGQPENNYKTTPPVLDSDGSFFLYSRLTVDKSRWQEGNVFSCSVMHEALHNHYTQKSLSLSLGKASGSAPAPAPEEEPCA

SEQ ID NO: 178 - protein, 300 aa, Artificial Sequence
  GLP-1 fusion 66
HGEGTFTSDLSKQMEEEAVRLFIEWLKNGGPSSGAPPPSGGGGSGGGGSGGGGSAESKYGPPCPPCPAPEAAGGPSVFLFPPKPKDTLMISRTPEVTCVVVDVSQEDPEVQFNWYVDGVEVHNAKTKPREEQFNSTYRVVSVLTVLHQDWLNGKEYKCKVSNKGLPSSIEKTISKAKGQPREPQVYTLPPSQEEMTKNQVSLTCLVKGFYPSDIAVEWESNGQPENNYKTTPPVLDSDGSFFLYSRLTVDKSRWQEGNVFSCSVMHEALHNHYTQKSLSLSLGKASGSAPAPAPEEEPCA

SEQ ID NO: 179 - protein, 289 aa, Artificial Sequence
  GLP-1 fusion 67
HGEGTFTSDLSKQMEEEAVRLFIEWLKNGGGGSGGGGSGGGGSAESKYGPPCPPCPAPEAAGGPSVFLFPPKPKDTLMISRTPEVTCVVVDVSQEDPEVQFNWYVDGVEVHNAKTKPREEQFNSTYRVVSVLTVLHQDWLNGKEYKCKVSNKGLPSSIEKTISKAKGQPREPQVYTLPPSQEEMTKNQVSLTCLVKGFYPSDIAVEWESNGQPENNYKTTPPVLDSDGSFFLYSRLTVDKSRWQEGNVFSCSVMHEALHNHYTQKSLSLSLGKASGSAPAPAPEEEPCA

SEQ ID NO: 180 - protein, 290 aa, Artificial Sequence; identical to SEQ ID NO: 132
  GLP-1 fusion 68

SEQ ID NO: 181 - protein, 285 aa, Artificial Sequence
  GLP-1 fusion 69
HGEGTFTSDVSSYLEEQAAKEFIAWLVKGGGGGGGGGGGGGGGGGGAESKYGPPCPPCPAPEAAGGPSVFLFPPKPKDTLMISRTPEVTCVVVDVSQEDPEVQFNWYVDGVEVHNAKTKPREEQFNSTYRVVSVLTVLHQDWLNGKEYKCKVSNKGLPSSIEKTISKAKGQPREPQVYTLPPSQEEMTKNQVSLTCLVKGFYPSDIAVEWESNGQPENNYKTTPPVLDSDGSFFLYSRLTVDKSRWQEGNVFSCSVMHEALHNHYTQKSLSLSLGKAPAPEEPCA

SEQ ID NO: 182 - protein, 285 aa, Artificial Sequence
  GLP-1 fusion 70
HGEGTFTSDVSSYLEEQAAKEFIAWLVKGGGGGGGAGGGGAGGGGAAESKYGPPCPPCPAPEAAGGPSVFLFPPKPKDTLMISRTPEVTCVVVDVSQEDPEVQFNWYVDGVEVHNAKTKPREEQFNSTYRVVSVLTVLHQDWLNGKEYKCKVSNKGLPSSIEKTISKAKGQPREPQVYTLPPSQEEMTKNQVSLTCLVKGFYPSDIAVEWESNGQPENNYKTTPPVLDSDGSFFLYSRLTVDKSRWQEGNVFSCSVMHEALHNHYTQKSLSLSLGKAPAPEEPCA

SEQ ID NO: 183 - protein, 293 aa, Artificial Sequence
  GLP-1 fusion 71
HGEGTFTSDLSKQMEEEAVRLFIEWLKNGGPSSGAPPPSGGGGGGGGGGGGGGGAESKYGPPCPPCPAPEAAGGPSVFLFPPKPKDTLMISRTPEVTCVVVDVSQEDPEVQFNWYVDGVEVHNAKTKPREEQFNSTYRVVSVLTVLHQDWLNGKEYKCKVSNKGLPSSIEKTISKAKGQPREPQVYTLPPSQEEMTKNQVSLTCLVKGFYPSDIAVEWESNGQPENNYKTTPPVLDSDGSFFLYSRLTVDKSRWQEGNVFSCSVMHEALHNHYTQKSLSLSLGKAPAPEEPCA

SEQ ID NO: 184 - protein, 293 aa, Artificial Sequence
  GLP-1 fusion 72
HGEGTFTSDLSKQMEEEAVRLFIEWLKNGGPSSGAPPPSGGGGAGGGGAGGGGAAESKYGPPCPPCPAPEAAGGPSVFLFPPKPKDTLMISRTPEVTCVVVDVSQEDPEVQFNWYVDGVEVHNAKTKPREEQFNSTYRVVSVLTVLHQDWLNGKEYKCKVSNKGLPSSIEKTISKAKGQPREPQVYTLPPSQEEMTKNQVSLTCLVKGFYPSDIAVEWESNGQPENNYKTTPPVLDSDGSFFLYSRLTVDKSRWQEGNVFSCSVMHEALHNHYTQKSLSLSLGKAPAPEEPCA

SEQ ID NO: 185 - protein, 289 aa, Artificial Sequence
  GLP-1 fusion 73
HGEGTFTSDVSSYLEEQAAKEFIAWLVKGGGGGGGSGGGGSGGGGSAERKCCVECPPCPAPEAAGGPSVFLFPPKPKDTLMISRTPEVTCVVVDVSQEDPEVQFNWYVDGVEVHNAKTKPREEQFNSTYRVVSVLTVLHQDWLNGKEYKCKVSNKGLPSSIEKTISKAKGQPREPQVYTLPPSQEEMTKNQVSLTCLVKGFYPSDIAVEWESNGQPENNYKTTPPVLDSDGSFFLYSRLTVDKSRWQEGNVFSCSVMHEALHNHYTQKSLSLSLGAPAPAPAPAPAPCP

SEQ ID NO: 186 - protein, 289 aa, Artificial Sequence
  GLP-1 fusion 74
HGEGTFTSDVSSYLEEQAAKEFIAWLVKGGGGGGGAGGGGAGGGGAAERKCCVECPPCPAPEAAGGPSVFLFPPKPKDTLMISRTPEVTCVVVDVSQEDPEVQFNWYVDGVEVHNAKTKPREEQFNSTYRVVSVLTVLHQDWLNGKEYKCKVSNKGLPSSIEKTISKAKGQPREPQVYTLPPSQEEMTKNQVSLTCLVKGFYPSDIAVEWESNGQPENNYKTTPPVLDSDGSFFLYSRLTVDKSRWQEGNVFSCSVMHEALHNHYTQKSLSLSLGAPAPAPAPAPAPCP

SEQ ID NO: 187 - protein, 295 aa, Artificial Sequence
  GLP-1 fusion 75
HGEGTFTSDVSSYLEEQAAKEFIAWLVKGGGGGGGAGGGGAGGGGAGGGGAGGGGAAGPPCPPCPAPEAAGGPSVFLFPPKPKDTLMISRTPEVTCVVVDVSQEDPEVQFNWYVDGVEVHNAKTKPREEQFNSTYRVVSVLTVLHQDWLNGKEYKCKVSNKGLPSSIEKTISKAKGQPREPQVYTLPPSQEEMTKNQVSLTCLVKGFYPSDIAVEWESNGQPENNYKTTPPVLDSDGSFFLYSRLTVDKSRWQEGNVFSCSVMHEALHNHYTQKSLSLSLGAPAPAPAPAPAPCP

SEQ ID NO: 188 - protein, 294 aa, Artificial Sequence
  GLP-1 fusion 76
HGEGTFTSDVSSYLEEQAAKEFIAWLVKGGGGGGGPGGGGPGGGGPGGGGPAESKYGPPCPPCPAPEAAGGPSVFLFPPKPKDTLMISRTPEVTCVVVDVSQEDPEVQFNWYVDGVEVHNAKTKPREEQFNSTYRVVSVLTVLHQDWLNGKEYKCKVSNKGLPSSIEKTISKAKGQPREPQVYTLPPSQEEMTKNQVSLTCLVKGFYPSDIAVEWESNGQPENNYKTTPPVLDSDGSFFLYSRLTVDKSRWQEGNVFSCSVMHEALHNHYTQKSLSLSLGAPAPAPAPAPAPCP

SEQ ID NO: 189 - protein, 294 aa, Artificial Sequence
  GLP-1 fusion 77
HGEGTFTSDVSSYLEEQAAKEFIAWLVKGGGGGGGHGGGGHGGGGHGGGGHAESKYGPPCPPCPAPEAAGGPSVFLFPPKPKDTLMISRTPEVTCVVVDVSQEDPEVQFNWYVDGVEVHNAKTKPREEQFNSTYRVVSVLTVLHQDWLNGKEYKCKVSNKGLPSSIEKTISKAKGQPREPQVYTLPPSQEEMTKNQVSLTCLVKGFYPSDIAVEWESNGQPENNYKTTPPVLDSDGSFFLYSRLTVDKSRWQEGNVFSCSVMHEALHNHYTQKSLSLSLGAPAPAPAPAPAPCP

SEQ ID NO: 190 - protein, 294 aa, Artificial Sequence
  GLP-1 fusion 78
HGEGTFTSDVSSYLEEQAAKEFIAWLVKGGGGGGGAGGGGAGGGGAGGGGAAESKYGPPCPPCPAPEAAGGPSVFLFPPKPKDTLMISRTPEVTCVVVDVSQEDPEVQFNWYVDGVEVHNAKTKPREEQFNSTYRVVSVLTVLHQDWLNGKEYKCKVSNKGLPSSIEKTISKAKGQPREPQVYTLPPSQEEMTKNQVSLTCLVKGFYPSDIAVEWESNGQPENNYKTTPPVLDSDGSFFLYSRLTVDKSRWQEGNVFSCSVMHEALHNHYTQKSLSLSLGAPAPAPAPAPAPCP

SEQ ID NO: 191 - protein, 311 aa, Artificial Sequence
  GLP-1 fusion 79
HGEGTFTSDVSSYLEEQAAKEFIAWLVKGGGASGGGGSGGGGSGGGGSGGGGSGGGGSGGGGSGGGGSGGGGSCPPCPAPEAAGGPSVFLFPPKPKDTLMISRTPEVTCVVVDVSQEDPEVQFNWYVDGVEVHNAKTKPREEQFNSTYRVVSVLTVLHQDWLNGKEYKCKVSNKGLPSSIEKTISKAKGQPREPQVYTLPPSQEEMTKNQVSLTCLVKGFYPSDIAVEWESNGQPENNYKTTPPVLDSDGSFFLYSRLTVDKSRWQEGNVFSCSVMHEALHNHYTQKSLSLSLGKASGSAPAPAPEEEPCA

SEQ ID NO: 192 - protein, 285 aa, Artificial Sequence
  GLP-1 fusion 80
HGEGTFTSDLSKQMEEEAVRLFIEWLKNGGPSSGAPPPSASGGGGSGGGGSCPPCPAPEAAGGPSVFLFPPKPKDTLMISRTPEVTCVVVDVSQEDPEVQFNWYVDGVEVHNAKTKPREEQFNSTYRVVSVLTVLHQDWLNGKEYKCKVSNKGLPSSIEKTISKAKGQPREPQVYTLPPSQEEMTKNQVSLTCLVKGFYPSDIAVEWESNGQPENNYKTTPPVLDSDGSFFLYSRLTVDKSRWQEGNVFSCSVMHEALHNHYTQKSLSLSLGKGGGGSGGGGSCA

SEQ ID NO: 193 - protein, 291 aa, Artificial Sequence
  GLP-1 fusion 81
HGEGTFTSDVSSYLEEQAAKEFIAWLVKGGGGGGGAGGGGAGGGGAAESKYGPPCPPCPAPEAAGGPSVFLFPPKPKDTLMISRTPEVTCVVVDVSQEDPEVQFNWYVDGVEVHNAKTKPREEQFNSTYRVVSVLTVLHQDWLNGKEYKCKVSNKGLPSSIEKTISKAKGQPREPQVYTLPPSQEEMTKNQVSLTCLVKGFYPSDIAVEWESNGQPENNYKTTPPVLDSDGSFFLYSRLTVDKSRWQEGNVFSCSVMHEALHNHYTQKSLSLSLGKGGGAPAPAPEEEPCA

SEQ ID NO: 194 - protein, 292 aa, Artificial Sequence
  GLP-1 fusion 82
HGEGTFTSDVSSYLEEQAAKEFIAWLVKGGGGGGGAGGGGAGGGGAAESKYGPPCPPCPAPEAAGGPSVFLFPPKPKDTLMISRTPEVTCVVVDVSQEDPEVQFNWYVDGVEVHNAKTKPREEQFNSTYRVVSVLTVLHQDWLNGKEYKCKVSNKGLPSSIEKTISKAKGQPREPQVYTLPPSQEEMTKNQVSLTCLVKGFYPSDIAVEWESNGQPENNYKTTPPVLDSDGSFFLYSRLTVDKSRWQEGNVFSCSVMHEALHNHYTQKSLSLSLGKASGSAPAPAPEEEPCA

SEQ ID NO: 195 - protein, 292 aa, Artificial Sequence
  GLP-1 fusion 83
HGEGTFTSDVSSYLEEQAAKEFIAWLVKGGGGGGGGGGGGGGGGGGAESKYGPPCPPCPAPEAAGGPSVFLFPPKPKDTLMISRTPEVTCVVVDVSQEDPEVQFNWYVDGVEVHNAKTKPREEQFNSTYRVVSVLTVLHQDWLNGKEYKCKVSNKGLPSSIEKTISKAKGQPREPQVYTLPPSQEEMTKNQVSLTCLVKGFYPSDIAVEWESNGQPENNYKTTPPVLDSDGSFFLYSRLTVDKSRWQEGNVFSCSVMHEALHNHYTQKSLSLSLGKASGSAPAPAPEEEPCA

SEQ ID NO: 196 - protein, 291 aa, Artificial Sequence
  GLP-1 fusion 84
HGEGTFTSDVSSYLEEQAAKEFIAWLVKGGGGGGGGGGGGGGGGGGAESKYGPPCPPCPAPEAAGGPSVFLFPPKPKDTLMISRTPEVTCVVVDVSQEDPEVQFNWYVDGVEVHNAKTKPREEQFNSTYRVVSVLTVLHQDWLNGKEYKCKVSNKGLPSSIEKTISKAKGQPREPQVYTLPPSQEEMTKNQVSLTCLVKGFYPSDIAVEWESNGQPENNYKTTPPVLDSDGSFFLYSRLTVDKSRWQEGNVFSCSVMHEALHNHYTQKSLSLSLGKGGGAPAPAPEEEPCA

SEQ ID NO: 197 - protein, 289 aa, Artificial Sequence
  GLP-1 fusion 85
HGEGTFTSDVSSYLEEQAAKEFIAWLVKGGGGGGGPGGGGPGGGGPAERKCCVECPPCPAPEAAGGPSVFLFPPKPKDTLMISRTPEVTCVVVDVSQEDPEVQFNWYVDGVEVHNAKTKPREEQFNSTYRVVSVLTVLHQDWLNGKEYKCKVSNKGLPSSIEKTISKAKGQPREPQVYTLPPSQEEMTKNQVSLTCLVKGFYPSDIAVEWESNGQPENNYKTTPPVLDSDGSFFLYSRLTVDKSRWQEGNVFSCSVMHEALHNHYTQKSLSLSLGAPAPAPAPAPAPCP

SEQ ID NO: 198 - protein, 289 aa, Artificial Sequence
  GLP-1 fusion 86
HGEGTFTSDVSSYLEEQAAKEFIAWLVKGGGGGGGHGGGGHGGGGHAERKCCVECPPCPAPEAAGGPSVFLFPPKPKDTLMISRTPEVTCVVVDVSQEDPEVQFNWYVDGVEVHNAKTKPREEQFNSTYRVVSVLTVLHQDWLNGKEYKCKVSNKGLPSSIEKTISKAKGQPREPQVYTLPPSQEEMTKNQVSLTCLVKGFYPSDIAVEWESNGQPENNYKTTPPVLDSDGSFFLYSRLTVDKSRWQEGNVFSCSVMHEALHNHYTQKSLSLSLGAPAPAPAPAPAPCP

SEQ ID NO: 199 - protein, 295 aa, Artificial Sequence
  GLP-1 fusion 87
HGEGTFTSDVSSYLEEQAAKEFIAWLVKGGGGGGGPGGGGPGGGGPGGGGPGGGGPAGPPCPPCPAPEAAGGPSVFLFPPKPKDTLMISRTPEVTCVVVDVSQEDPEVQFNWYVDGVEVHNAKTKPREEQFNSTYRVVSVLTVLHQDWLNGKEYKCKVSNKGLPSSIEKTISKAKGQPREPQVYTLPPSQEEMTKNQVSLTCLVKGFYPSDIAVEWESNGQPENNYKTTPPVLDSDGSFFLYSRLTVDKSRWQEGNVFSCSVMHEALHNHYTQKSLSLSLGAPAPAPAPAPAPCP

SEQ ID NO: 200 - protein, 295 aa, Artificial Sequence
  GLP-1 fusion 88
HGEGTFTSDVSSYLEEQAAKEFIAWLVKGGGGGGGHGGGGHGGGGHGGGGHGGGGHAGPPCPPCPAPEAAGGPSVFLFPPKPKDTLMISRTPEVTCVVVDVSQEDPEVQFNWYVDGVEVHNAKTKPREEQFNSTYRVVSVLTVLHQDWLNGKEYKCKVSNKGLPSSIEKTISKAKGQPREPQVYTLPPSQEEMTKNQVSLTCLVKGFYPSDIAVEWESNGQPENNYKTTPPVLDSDGSFFLYSRLTVDKSRWQEGNVFSCSVMHEALHNHYTQKSLSLSLGAPAPAPAPAPAPCP

SEQ ID NO: 201 - protein, 292 aa, Artificial Sequence
  GLP-1 fusion 89
HGEGTFTSDVSSYLEEQAAKEFIAWLVKGGGGGGGSGGGGSGGGGSAERKCCVECPPCPAPEAAGGPSVFLFPPKPKDTLMISRTPEVTCVVVDVSQEDPEVQFNWYVDGVEVHNAKTKPREEQFNSTYRVVSVLTVLHQDWLNGKEYKCKVSNKGLPSSIEKTISKAKGQPREPQVYTLPPSQEEMTKNQVSLTCLVKGFYPSDIAVEWESNGQPENNYKTTPPVLDSDGSFFLYSRLTVDKSRWQEGNVFSCSVMHEALHNHYTQKSLSLSLGAPAPAPAPAPAPCPEEP

SEQ ID NO: 202 - protein, 292 aa, Artificial Sequence
  GLP-1 fusion 90
HGEGTFTSDVSSYLEEQAAKEFIAWLVKGGGGGGGPGGGGPGGGGPAERKCCVECPPCPAPEAAGGPSVFLFPPKPKDTLMISRTPEVTCVVVDVSQEDPEVQFNWYVDGVEVHNAKTKPREEQFNSTYRVVSVLTVLHQDWLNGKEYKCKVSNKGLPSSIEKTISKAKGQPREPQVYTLPPSQEEMTKNQVSLTCLVKGFYPSDIAVEWESNGQPENNYKTTPPVLDSDGSFFLYSRLTVDKSRWQEGNVFSCSVMHEALHNHYTQKSLSLSLGAPAPAPAPAPAPCPEEP

SEQ ID NO: 203 - protein, 292 aa, Artificial Sequence
  GLP-1 fusion 91
HGEGTFTSDVSSYLEEQAAKEFIAWLVKGGGGGGGHGGGGHGGGGHAERKCCVECPPCPAPEAAGGPSVFLFPPKPKDTLMISRTPEVTCVVVDVSQEDPEVQFNWYVDGVEVHNAKTKPREEQFNSTYRVVSVLTVLHQDWLNGKEYKCKVSNKGLPSSIEKTISKAKGQPREPQVYTLPPSQEEMTKNQVSLTCLVKGFYPSDIAVEWESNGQPENNYKTTPPVLDSDGSFFLYSRLTVDKSRWQEGNVFSCSVMHEALHNHYTQKSLSLSLGAPAPAPAPAPAPCPEEP

SEQ ID NO: 204 - protein, 292 aa, Artificial Sequence
  GLP-1 fusion 92
HGEGTFTSDVSSYLEEQAAKEFIAWLVKGGGGGGGAGGGGAGGGGAAERKCCVECPPCPAPEAAGGPSVFLFPPKPKDTLMISRTPEVTCVVVDVSQEDPEVQFNWYVDGVEVHNAKTKPREEQFNSTYRVVSVLTVLHQDWLNGKEYKCKVSNKGLPSSIEKTISKAKGQPREPQVYTLPPSQEEMTKNQVSLTCLVKGFYPSDIAVEWESNGQPENNYKTTPPVLDSDGSFFLYSRLTVDKSRWQEGNVFSCSVMHEALHNHYTQKSLSLSLGAPAPAPAPAPAPCPEEP

SEQ ID NO: 205 - protein, 298 aa, Artificial Sequence
  GLP-1 fusion 93
HGEGTFTSDVSSYLEEQAAKEFIAWLVKGGGGGGGPGGGGPGGGGPGGGGPGGGGPAGPPCPPCPAPEAAGGPSVFLFPPKPKDTLMISRTPEVTCVVVDVSQEDPEVQFNWYVDGVEVHNAKTKPREEQFNSTYRVVSVLTVLHQDWLNGKEYKCKVSNKGLPSSIEKTISKAKGQPREPQVYTLPPSQEEMTKNQVSLTCLVKGFYPSDIAVEWESNGQPENNYKTTPPVLDSDGSFFLYSRLTVDKSRWQEGNVFSCSVMHEALHNHYTQKSLSLSLGAPAPAPAPAPAPCPEEP

SEQ ID NO: 206 - protein, 298 aa, Artificial Sequence
  GLP-1 fusion 94
HGEGTFTSDVSSYLEEQAAKEFIAWLVKGGGGGGGHGGGGHGGGGHGGGGHGGGGHAGPPCPPCPAPEAAGGPSVFLFPPKPKDTLMISRTPEVTCVVVDVSQEDPEVQFNWYVDGVEVHNAKTKPREEQFNSTYRVVSVLTVLHQDWLNGKEYKCKVSNKGLPSSIEKTISKAKGQPREPQVYTLPPSQEEMTKNQVSLTCLVKGFYPSDIAVEWESNGQPENNYKTTPPVLDSDGSFFLYSRLTVDKSRWQEGNVFSCSVMHEALHNHYTQKSLSLSLGAPAPAPAPAPAPCPEEP

SEQ ID NO: 207 - protein, 298 aa, Artificial Sequence
  GLP-1 fusion 95
HGEGTFTSDVSSYLEEQAAKEFIAWLVKGGGGGGGAGGGGAGGGGAGGGGAGGGGAAGPPCPPCPAPEAAGGPSVFLFPPKPKDTLMISRTPEVTCVVVDVSQEDPEVQFNWYVDGVEVHNAKTKPREEQFNSTYRVVSVLTVLHQDWLNGKEYKCKVSNKGLPSSIEKTISKAKGQPREPQVYTLPPSQEEMTKNQVSLTCLVKGFYPSDIAVEWESNGQPENNYKTTPPVLDSDGSFFLYSRLTVDKSRWQEGNVFSCSVMHEALHNHYTQKSLSLSLGAPAPAPAPAPAPCPEEP

SEQ ID NO: 208 - protein, 297 aa, Artificial Sequence
  GLP-1 fusion 96
HGEGTFTSDVSSYLEEQAAKEFIAWLVKGGGGGGGPGGGGPGGGGPGGGGPAESKYGPPCPPCPAPEAAGGPSVFLFPPKPKDTLMISRTPEVTCVVVDVSQEDPEVQFNWYVDGVEVHNAKTKPREEQFNSTYRVVSVLTVLHQDWLNGKEYKCKVSNKGLPSSIEKTISKAKGQPREPQVYTLPPSQEEMTKNQVSLTCLVKGFYPSDIAVEWESNGQPENNYKTTPPVLDSDGSFFLYSRLTVDKSRWQEGNVFSCSVMHEALHNHYTQKSLSLSLGAPAPAPAPAPAPCPEEP

SEQ ID NO: 209 - protein, 297 aa, Artificial Sequence
  GLP-1 fusion 97
HGEGTFTSDVSSYLEEQAAKEFIAWLVKGGGGGGGHGGGGHGGGGHGGGGHAESKYGPPCPPCPAPEAAGGPSVFLFPPKPKDTLMISRTPEVTCVVVDVSQEDPEVQFNWYVDGVEVHNAKTKPREEQFNSTYRVVSVLTVLHQDWLNGKEYKCKVSNKGLPSSIEKTISKAKGQPREPQVYTLPPSQEEMTKNQVSLTCLVKGFYPSDIAVEWESNGQPENNYKTTPPVLDSDGSFFLYSRLTVDKSRWQEGNVFSCSVMHEALHNHYTQKSLSLSLGAPAPAPAPAPAPCPEEP

SEQ ID NO: 210 - protein, 297 aa, Artificial Sequence
  GLP-1 fusion 98
HGEGTFTSDVSSYLEEQAAKEFIAWLVKGGGGGGGAGGGGAGGGGAGGGGAAESKYGPPCPPCPAPEAAGGPSVFLFPPKPKDTLMISRTPEVTCVVVDVSQEDPEVQFNWYVDGVEVHNAKTKPREEQFNSTYRVVSVLTVLHQDWLNGKEYKCKVSNKGLPSSIEKTISKAKGQPREPQVYTLPPSQEEMTKNQVSLTCLVKGFYPSDIAVEWESNGQPENNYKTTPPVLDSDGSFFLYSRLTVDKSRWQEGNVFSCSVMHEALHNHYTQKSLSLSLGAPAPAPAPAPAPCPEEP

SEQ ID NO: 211 - protein, 294 aa, Artificial Sequence
  GLP-1 fusion 99
HGEGTFTSDVSSYLEEQAAKEFIAWLVKGGGPAPAPAPAPAPAPAPAPAPAPESKYGPPCPPCPAPEAAGGPSVFLFPPKPKDTLMISRTPEVTCVVVDVSQEDPEVQFNWYVDGVEVHNAKTKPREEQFNSTYRVVSVLTVLHQDWLNGKEYKCKVSNKGLPSSIEKTISKAKGQPREPQVYTLPPSQEEMTKNQVSLTCLVKGFYPSDIAVEWESNGQPENNYKTTPPVLDSDGSFFLYSRLTVDKSRWQEGNVFSCSVMHEALHNHYTQKSLSLSLGAPAPAPAPAPAPCP

SEQ ID NO: 212 - protein, 297 aa, Artificial Sequence
  GLP-1 fusion 100
HGEGTFTSDVSSYLEEQAAKEFIAWLVKGGGPAPAPAPAPAPAPAPAPAPAAESKYGPPCPPCPAPEAAGGPSVFLFPPKPKDTLMISRTPEVTCVVVDVSQEDPEVQFNWYVDGVEVHNAKTKPREEQFNSTYRVVSVLTVLHQDWLNGKEYKCKVSNKGLPSSIEKTISKAKGQPREPQVYTLPPSQEEMTKNQVSLTCLVKGFYPSDIAVEWESNGQPENNYKTTPPVLDSDGSFFLYSRLTVDKSRWQEGNVFSCSVMHEALHNHYTQKSLSLSLGAPAPAPAPAPAPCPEEP

SEQ ID NO: 213 - protein, 297 aa, Artificial Sequence
  GLP-1 fusion 101
HGEGTFTSDVSSYLEEQAAKEFIAWLVKGGGPAPAPAPAPAPAPAPAPAPAPESKYGPPCPPCPAPEAAGGPSVFLFPPKPKDTLMISRTPEVTCVVVDVSQEDPEVQFNWYVDGVEVHNAKTKPREEQFNSTYRVVSVLTVLHQDWLNGKEYKCKVSNKGLPSSIEKTISKAKGQPREPQVYTLPPSQEEMTKNQVSLTCLVKGFYPSDIAVEWESNGQPENNYKTTPPVLDSDGSFFLYSRLTVDKSRWQEGNVFSCSVMHEALHNHYTQKSLSLSLGAPAPAPAPAPAPCPEEP

SEQ ID NO: 214 - protein, 294 aa, Artificial Sequence
  GLP-1 fusion 102
HGEGTFTSDVSSYLEEQAAKEFIAWLVKGGGGGGGAGGGGAGGGGAGGGGAESKYGPPCPPCPAPEAAGGPSVFLFPPKPKDTLMISRTPEVTCVVVDVSQEDPEVQFNWYVDGVEVHNAKTKPREEQFNSTYRVVSVLTVLHQDWLNGKEYKCKVSNKGLPSSIEKTISKAKGQPREPQVYTLPPSQEEMTKNQVSLTCLVKGFYPSDIAVEWESNGQPENNYKTTPPVLDSDGSFFLYSRLTVDKSRWQEGNVFSCSVMHEALHNHYTQKSLSLSLGGGGAPAPAPEEEPCA

SEQ ID NO: 215 - protein, 289 aa, Artificial Sequence
  GLP-1 fusion 103
HGEGTFTSDVSSYLEEQAAKEFIAWLVKGGGGGGGAGGGGAGGGGAESKYGPPCPPCPAPEAAGGPSVFLFPPKPKDTLMISRTPEVTCVVVDVSQEDPEVQFNWYVDGVEVHNAKTKPREEQFNSTYRVVSVLTVLHQDWLNGKEYKCKVSNKGLPSSIEKTISKAKGQPREPQVYTLPPSQEEMTKNQVSLTCLVKGFYPSDIAVEWESNGQPENNYKTTPPVLDSDGSFFLYSRLTVDKSRWQEGNVFSCSVMHEALHNHYTQKSLSLSLGGGGAPAPAPEEEPCA

SEQ ID NO: 216 - protein, 288 aa, Artificial Sequence
  GLP-1 fusion 104
HGEGTFTSDLSKQMEEEAVRLFIEWLKNGGGGSGGGGSGGGGSAESKYGPPCPPCPAPEAAGGPSVFLFPPKPKDTLMISRTPEVTCVVVDVSQEDPEVQFNWYVDGVEVHNAKTKPREEQFNSTYRVVSVLTVLHQDWLNGKEYKCKVSNKGLPSSIEKTISKAKGQPREPQVYTLPPSQEEMTKNQVSLTCLVKGFYPSDIAVEWESNGQPENNYKTTPPVLDSDGSFFLYSRLTVDKSRWQEGNVFSCSVMHEALHNHYTQKSLSLSLGKGGGAPAPAPEEEPCA

SEQ ID NO: 217 - protein, 287 aa, Artificial Sequence
  GLP-1 fusion 105
HGEGTFTSDLSKQMEEEAVRLFIEWLKNGGGGSGGGGSGGGGSAESKYGPPCPPCPAPEAAGGPSVFLFPPKPKDTLMISRTPEVTCVVVDVSQEDPEVQFNWYVDGVEVHNAKTKPREEQFNSTYRVVSVLTVLHQDWLNGKEYKCKVSNKGLPSSIEKTISKAKGQPREPQVYTLPPSQEEMTKNQVSLTCLVKGFYPSDIAVEWESNGQPENNYKTTPPVLDSDGSFFLYSRLTVDKSRWQEGNVFSCSVMHEALHNHYTQKSLSLSLGGGGAPAPAPEEEPCA

SEQ ID NO: 218 - protein, 289 aa, Artificial Sequence
  GLP-1 fusion 106
HGEGTFTSDLSKQMEEEAVRLFIEWLKNGGGGSGGGGSGGGGSAESKYGPPCPPCPAPEAAGGPSVFLFPPKPKDTLMISRTPEVTCVVVDVSQEDPEVQFNWYVDGVEVHNAKTKPREEQFNSTYRVVSVLTVLHQDWLNGKEYKCKVSNKGLPSSIEKTISKAKGQPREPQVYTLPPSQEEMTKNQVSLTCLVKGFYPSDIAVEWESNGQPENNYKTTPPVLDSDGSFFLYSRLTVDKSRWQEGNVFSCSVMHEALHNHYTQKSLSLSLGGGGGGGGGGGGGGGGCA

SEQ ID NO: 219 - protein, 289 aa, Artificial Sequence
  GLP-1 fusion 107
HGEGTFTSDLSKQMEEEAVRLFIEWLKNGGGGSGGGGSGGGGSAESKYGPPCPPCPAPEAAGGPSVFLFPPKPKDTLMISRTPEVTCVVVDVSQEDPEVQFNWYVDGVEVHNAKTKPREEQFNSTYRVVSVLTVLHQDWLNGKEYKCKVSNKGLPSSIEKTISKAKGQPREPQVYTLPPSQEEMTKNQVSLTCLVKGFYPSDIAVEWESNGQPENNYKTTPPVLDSDGSFFLYSRLTVDKSRWQEGNVFSCSVMHEALHNHYTQKSLSLSLGGGGGAGGGGAGGGGACA

SEQ ID NO: 220 - protein, 286 aa, Artificial Sequence
  GLP-1 fusion 108
HGEGTFTSDLSKQMEEEAVRLFIEWLKNGGGGSGGGGSGGGGSAESKYGPPCPPCPAPEAAGGPSVFLFPPKPKDTLMISRTPEVTCVVVDVSQEDPEVQFNWYVDGVEVHNAKTKPREEQFNSTYRVVSVLTVLHQDWLNGKEYKCKVSNKGLPSSIEKTISKAKGQPREPQVYTLPPSQEEMTKNQVSLTCLVKGFYPSDIAVEWESNGQPENNYKTTPPVLDSDGSFFLYSRLTVDKSRWQEGNVFSCSVMHEALHNHYTQKSLSLSLGAPAPAPAPAPAPCP

SEQ ID NO: 221 - protein, 289 aa, Artificial Sequence
  GLP-1 fusion 109
HGEGTFTSDLSKQMEEEAVRLFIEWLKNGGGGSGGGGSGGGGSAESKYGPPCPPCPAPEAAGGPSVFLFPPKPKDTLMISRTPEVTCVVVDVSQEDPEVQFNWYVDGVEVHNAKTKPREEQFNSTYRVVSVLTVLHQDWLNGKEYKCKVSNKGLPSSIEKTISKAKGQPREPQVYTLPPSQEEMTKNQVSLTCLVKGFYPSDIAVEWESNGQPENNYKTTPPVLDSDGSFFLYSRLTVDKSRWQEGNVFSCSVMHEALHNHYTQKSLSLSLGAPAPAPAPAPAPCPEEP

SEQ ID NO: 222 - protein, 288 aa, Artificial Sequence
  GLP-1 fusion 110
HGEGTFTSDLSKQMEEEAVRLFIEWLKNGGGGAGGGGAGGGGAAESKYGPPCPPCPAPEAAGGPSVFLFPPKPKDTLMISRTPEVTCVVVDVSQEDPEVQFNWYVDGVEVHNAKTKPREEQFNSTYRVVSVLTVLHQDWLNGKEYKCKVSNKGLPSSIEKTISKAKGQPREPQVYTLPPSQEEMTKNQVSLTCLVKGFYPSDIAVEWESNGQPENNYKTTPPVLDSDGSFFLYSRLTVDKSRWQEGNVFSCSVMHEALHNHYTQKSLSLSLGKGGGAPAPAPEEEPCA

SEQ ID NO: 223 - protein, 289 aa, Artificial Sequence
  GLP-1 fusion 111
HGEGTFTSDLSKQMEEEAVRLFIEWLKNGGGGAGGGGAGGGGAAESKYGPPCPPCPAPEAAGGPSVFLFPPKPKDTLMISRTPEVTCVVVDVSQEDPEVQFNWYVDGVEVHNAKTKPREEQFNSTYRVVSVLTVLHQDWLNGKEYKCKVSNKGLPSSIEKTISKAKGQPREPQVYTLPPSQEEMTKNQVSLTCLVKGFYPSDIAVEWESNGQPENNYKTTPPVLDSDGSFFLYSRLTVDKSRWQEGNVFSCSVMHEALHNHYTQKSLSLSLGGGGGGGGGGGGGGGGCA

SEQ ID NO: 224 - protein, 292 aa, Artificial Sequence
  GLP-1 fusion 112
HGEGTFTSDVSSYLEEQAAKEFIAWLVKGGGGGGGAGGGGAGGGGAAESKYGPPCPPCPAPEAAGGPSVFLFPPKPKDTLMISRTPEVTCVVVDVSQEDPEVQFNWYVDGVEVHNAKTKPREEQFNSTYRVVSVLTVLHQDWLNGKEYKCKVSNKGLPSSIEKTISKAKGQPREPQVYTLPPSQEEMTKNQVSLTCLVKGFYPSDIAVEWESNGQPENNYKTTPPVLDSDGSFFLYSRLTVDKSRWQEGNVFSCSVMHEALHNHYTQKSLSLSLGGGGGGGGGGGGGGGGCA

SEQ ID NO: 225 - protein, 35 aa, Artificial Sequence; identical to SEQ ID NO: 27
  GLP-1 fusion coupled cyclic PYY peptide conjugate
  Gly (1)..(1): Gly with a cyclic modification
  Lys (10)..(10): Lys with a GLP-1 fusion 1 chemical modification
  Cys (29)..(29): Cys with a cyclic modification
  Arg (34)..(34): Arg with a N-Me chemical modification

SEQ ID NO: 226 - protein, 35 aa, Artificial Sequence; identical to SEQ ID NO: 20
  GLP-1 fusion coupled cyclic PYY peptide conjugate
  Ala (1)..(1): Ala, wherein the alanine is a beta-alanine with a cyclic modification
  Lys (10)..(10): Lys with a GLP-1 fusion 1 chemical modification
  Cys (29)..(29): Cys with a cyclic modification
  Arg (34)..(34): Arg with a N-Me chemical modification

SEQ ID NO: 227 - protein, 35 aa, Artificial Sequence; identical to SEQ ID NO: 20
  GLP-1 fusion coupled cyclic PYY peptide conjugate
  Ala (1)..(1): Ala, wherein the alanine is a beta-alanine with a cyclic modification
  Lys (10)..(10): Lys with a GLP-1 fusion 1 chemical modification
  Cys (29)..(29): Cys with a cyclic modification
  Arg (34)..(34): Arg with a psi-(R35, Y36) chemical modification
  Tyr (35)..(35): Tyr with a psi-(R35, Y36) chemical modification

SEQ ID NO: 228 - protein, 35 aa, Artificial Sequence; identical to SEQ ID NO: 18
  GLP-1 fusion coupled cyclic PYY peptide conjugate
  Gly (1)..(1): Gly with a cyclic modification
  Lys (10)..(10): Lys with a GLP-1 fusion 1 chemical modification
  Cys (29)..(29): Cys with a cyclic modification
  Arg (34)..(34): Arg with a psi-(R35, Y36) chemical modification
  Tyr (35)..(35): Tyr with a psi-(R35, Y36) chemical modification

SEQ ID NO: 229 - protein, 35 aa, Artificial Sequence; identical to SEQ ID NO: 27
  GLP-1 fusion coupled cyclic PYY peptide conjugate
  Gly (1)..(1): Gly with a cyclic modification
  Lys (10)..(10): Lys with a GLP-1 fusion 24 chemical modification
  Cys (29)..(29): Cys with a cyclic modification
  Arg (34)..(34): Arg with a N-Me chemical modification

SEQ ID NO: 230 - protein, 35 aa, Artificial Sequence; identical to SEQ ID NO: 20
  GLP-1 fusion coupled cyclic PYY peptide conjugate
  Ala (1)..(1): Ala, wherein the alanine is a beta-alanine with a cyclic modification
  Lys (10)..(10): Lys with a GLP-1 fusion 24 chemical modification
  Cys (29)..(29): Cys with a cyclic modification
  Arg (34)..(34): Arg with a N-Me chemical modification

SEQ ID NO: 231 - protein, 35 aa, Artificial Sequence; identical to SEQ ID NO: 20
  GLP-1 fusion coupled cyclic PYY peptide conjugate
  Ala (1)..(1): Ala, wherein the alanine is a beta-alanine with a cyclic modification
  Lys (10)..(10): Lys with a GLP-1 fusion 24 chemical modification
  Cys (29)..(29): Cys with a cyclic modification
  Arg (34)..(34): Arg with a psi-(R35, Y36) chemical modification
  Tyr (35)..(35): Tyr with a psi-(R35, Y36) chemical modification

SEQ ID NO: 232 - protein, 35 aa, Artificial Sequence; identical to SEQ ID NO: 18
  GLP-1 fusion coupled cyclic PYY peptide conjugate
  Gly (1)..(1): Gly with a cyclic modification
  Lys (10)..(10): Lys with a GLP-1 fusion 24 chemical modification
  Cys (29)..(29): Cys with a cyclic modification
  Arg (34)..(34): Arg with a psi-(R35, Y36) chemical modification
  Tyr (35)..(35): Tyr with a psi-(R35, Y36) chemical modification

SEQ ID NO: 233 - protein, 35 aa, Artificial Sequence; identical to SEQ ID NO: 27
  GLP-1 fusion coupled cyclic PYY peptide conjugate
  Gly (1)..(1): Gly with a cyclic modification
  Lys (10)..(10): Lys with a GLP-1 fusion 70 chemical modification
  Cys (29)..(29): Cys with a cyclic modification
  Arg (34)..(34): Arg with a N-Me chemical modification

SEQ ID NO: 234 - protein, 35 aa, Artificial Sequence; identical to SEQ ID NO: 27
  GLP-1 fusion coupled cyclic PYY peptide conjugate
  Gly (1)..(1): Gly with a cyclic modification
  Lys (10)..(10): Lys with a GLP-1 fusion 11 chemical modification
  Cys (29)..(29): Cys with a cyclic modification
  Arg (34)..(34): Arg with a N-Me chemical modification

SEQ ID NO: 235 - protein, 35 aa, Artificial Sequence; identical to SEQ ID NO: 27
  GLP-1 fusion coupled cyclic PYY peptide conjugate
  Gly (1)..(1): Gly with a cyclic modification
  Lys (10)..(10): Lys with a GLP-1 fusion 28 chemical modification
  Cys (29)..(29): Cys with a cyclic modification
  Arg (34)..(34): Arg with a N-Me chemical modification

SEQ ID NO: 236 - protein, 35 aa, Artificial Sequence; identical to SEQ ID NO: 27
  GLP-1 fusion coupled cyclic PYY peptide conjugate
  Gly (1)..(1): Gly with a cyclic modification
  Lys (10)..(10): Lys with a GLP-1 fusion 67 chemical modification
  Cys (29)..(29): Cys with a cyclic modification
  Arg (34)..(34): Arg with a N-Me chemical modification

SEQ ID NO: 237 - protein, 35 aa, Artificial Sequence; identical to SEQ ID NO: 27
  GLP-1 fusion coupled cyclic PYY peptide conjugate
  Gly (1)..(1): Gly with a cyclic modification
  Lys (10)..(10): Lys with a GLP-1 fusion 27 chemical modification
  Cys (29)..(29): Cys with a cyclic modification
  Arg (34)..(34): Arg with a N-Me chemical modification

SEQ ID NO: 238 - protein, 35 aa, Artificial Sequence; identical to SEQ ID NO: 27
  GLP-1 fusion coupled cyclic PYY peptide conjugate
  Gly (1)..(1): Gly with a cyclic modification
  Lys (10)..(10): Lys with a GLP-1 fusion 23 chemical modification
  Cys (29)..(29): Cys with a cyclic modification
  Arg (34)..(34): Arg with a N-Me chemical modification

SEQ ID NO: 239 - protein, 35 aa, Artificial Sequence; identical to SEQ ID NO: 27
  GLP-1 fusion coupled cyclic PYY peptide conjugate
  Gly (1)..(1): Gly with a cyclic modification
  Lys (10)..(10): Lys with a GLP-1 fusion 54 chemical modification
  Cys (29)..(29): Cys with a chemical modification
  Arg (34)..(34): Arg with a N-Me chemical modification

SEQ ID NO: 240 - protein, 35 aa, Artificial Sequence; identical to SEQ ID NO: 27
  GLP-1 fusion coupled cyclic PYY peptide conjugate
  Gly (1)..(1): Gly with a cyclic modification
  Lys (10)..(10): Lys with a GLP-1 fusion 63 chemical modification
  Cys (29)..(29): Cys with a cyclic modification
  Arg (34)..(34): Arg with a N-Me chemical modification

SEQ ID NO: 241 - protein, 35 aa, Artificial Sequence; identical to SEQ ID NO: 27
  GLP-1 fusion coupled cyclic PYY peptide conjugate
  Gly (1)..(1): Gly with a cyclic modification
  Lys (10)..(10): Lys with a GLP-1 fusion 64 chemical modification
  Cys (29)..(29): Cys with a cyclic modification
  Arg (34)..(34): Arg with a N-Me chemical modification

SEQ ID NO: 242 - protein, 35 aa, Artificial Sequence; identical to SEQ ID NO: 27
  GLP-1 fusion coupled cyclic PYY peptide conjugate
  Gly (1)..(1): Gly with a cyclic modification
  Lys (10)..(10): Lys with a GLP-1 fusion 22 chemical modification
  Cys (29)..(29): Cys with a cyclic modification
  Arg (34)..(34): Arg with a N-Me chemical modification

SEQ ID NO: 243 - protein, 35 aa, Artificial Sequence; identical to SEQ ID NO: 27
  GLP-1 fusion coupled cyclic PYY peptide conjugate
  Gly (1)..(1): Gly with a cyclic modification
  Lys (10)..(10): Lys with a GLP-1 fusion 49 chemical modification
  Cys (29)..(29): Cys with a cyclic modification
  Arg (34)..(34): Arg with a N-Me chemical modification

SEQ ID NO: 244 - protein, 35 aa, Artificial Sequence; identical to SEQ ID NO: 1
  GLP-1 fusion coupled cyclic PYY peptide conjugate
  Ala (1)..(1): Ala, wherein the ala is a beta-alanine with a cyclic modification
  Lys (10)..(10): Lys with a PEG24 GLP-1 fusion 34 chemical modification
  Cys (30)..(30): Cys, wherein the cys is a homocysteine with a cyclic modification
  Arg (34)..(34): Arg with a psi-(R35, Y36) chemical modification
  Tyr (35)..(35): Tyr with a psi-(R35, Y36) chemical modification

SEQ ID NO: 245 - protein, 35 aa, Artificial Sequence; identical to SEQ ID NO: 27
  GLP-1 fusion coupled cyclic PYY peptide conjugate
  Gly (1)..(1): Gly with a cyclic modification
  Lys (10)..(10): Lys with a GLP-1 fusion 35 chemical modification
  Cys (29)..(29): Cys with a cyclic modification
  Arg (34)..(34): Arg with a N-Me chemical modification

SEQ ID NO: 246 - protein, 35 aa, Artificial Sequence; identical to SEQ ID NO: 27
  GLP-1 fusion coupled cyclic PYY peptide conjugate
  Gly (1)..(1): Gly with a cyclic modification
  Lys (10)..(10): Lys with a GLP-1 fusion 65 chemical modification
  Cys (29)..(29): Cys with a cyclic modification
  Arg (34)..(34): Arg with a N-Me chemical modification

SEQ ID NO: 247 - protein, 35 aa, Artificial Sequence; identical to SEQ ID NO: 27
  GLP-1 fusion coupled cyclic PYY peptide conjugate
  Gly (1)..(1): Gly with a cyclic modification
  Lys (10)..(10): Lys with a GLP-1 fusion 45 chemical modification
  Cys (29)..(29): Cys with a cyclic modification
  Arg (34)..(34): Arg with a N-Me chemical modification

SEQ ID NO: 248 - protein, 35 aa, Artificial Sequence; identical to SEQ ID NO: 27
  GLP-1 fusion coupled cyclic PYY peptide conjugate
  Gly (1)..(1): Gly with a cyclic modification
  Lys (10)..(10): Lys with a GLP-1 fusion 40 chemical modification
  Cys (29)..(29): Cys with a cyclic modification
  Arg (34)..(34): Arg with a N-Me chemical modification

SEQ ID NO: 249 - protein, 35 aa, Artificial Sequence
  GLP-1 fusion coupled cyclic PYY peptide conjugate
  Gly (1)..(1): Gly with a cyclic modification
  Lys (10)..(10): Lys with a GLP-1 fusion 40 chemical modification
  Glu (29)..(29): Glu with a cyclic modification
  Arg (34)..(34): Arg with a N-Me chemical modification
GIKPEAPGEKASPEELNRYYASLRHYLNEVTRQRY

SEQ ID NO: 250 - protein, 35 aa, Artificial Sequence; identical to SEQ ID NO: 24
  GLP-1 fusion coupled cyclic PYY peptide conjugate
  Gly (1)..(1): Gly with a cyclic modification
  Lys (10)..(10): Lys with a GLP-1 fusion 40 chemical modification
  Glu (29)..(29): Glu with a cyclic modification
  Arg (34)..(34): Arg with a psi-(R35, Y36) chemical modification
  Tyr (35)..(35): Tyr with a psi-(R35, Y36) chemical modification

SEQ ID NO: 251 - protein, 35 aa, Artificial Sequence; identical to SEQ ID NO: 27
  GLP-1 fusion coupled cyclic PYY peptide conjugate
  Gly (1)..(1): Gly with a cyclic modification
  Lys (10)..(10): Lys with a GLP-1 fusion 19 chemical modification
  Cys (29)..(29): Cys with a cyclic modification
  Arg (34)..(34): Arg with a N-Me chemical modification

SEQ ID NO: 252 - protein, 35 aa, Artificial Sequence; identical to SEQ ID NO: 27
  GLP-1 fusion coupled cyclic PYY peptide conjugate
  Gly (1)..(1): Gly with a cyclic modification
  Lys (10)..(10): Lys with a GLP-1 fusion 8 chemical modification
  Cys (29)..(29): Cys with a cyclic modification
  Arg (34)..(34): Arg with a N-Me chemical modification

SEQ ID NO: 253 - protein, 35 aa, Artificial Sequence; identical to SEQ ID NO: 34
  GLP-1 fusion coupled cyclic PYY peptide conjugate
  Xaa (1)..(1): Xaa is a gamma amino-butyric acid with a cyclic modification
  Lys (10)..(10): Lys with a GLP-1 fusion 34 chemical modification
  Cys (29)..(29): Cys, wherein cys is a homocysteine with a cyclic modification
  Arg (34)..(34): Arg with a N-Me chemical modification

SEQ ID NO: 254 - protein, 35 aa, Artificial Sequence; identical to SEQ ID NO: 27
  GLP-1 fusion coupled cyclic PYY peptide conjugate
  Gly (1)..(1): Gly with a cyclic modification
  Lys (10)..(10): Lys with a GLP-1 fusion 42 chemical modification
  Cys (29)..(29): Cys with a cyclic modification
  Arg (34)..(34): Arg with a N-Me chemical modification

SEQ ID NO: 255 - protein, 35 aa, Artificial Sequence; identical to SEQ ID NO: 27
  GLP-1 fusion coupled cyclic PYY peptide conjugate
  Gly (1)..(1): Gly with a cyclic modification
  Lys (10)..(10): Lys with a GLP-1 fusion 59 chemical modification
  Cys (29)..(29): Cys with a cyclic modification
  Arg (34)..(34): Arg with a N-Me chemical modification

SEQ ID NO: 256 - protein, 35 aa, Artificial Sequence; identical to SEQ ID NO: 27
  GLP-1 fusion coupled cyclic PYY peptide conjugate
  Gly (1)..(1): Gly with a cyclic modification
  Lys (10)..(10): Lys with a GLP-1 fusion 60 chemical modification
  Cys (29)..(29): Cys with a cyclic modification
  Arg (34)..(34): Arg with a N-Me chemical modification

SEQ ID NO: 257 - protein, 35 aa, Artificial Sequence; identical to SEQ ID NO: 27
  GLP-1 fusion coupled cyclic PYY peptide conjugate
  Gly (1)..(1): Gly with a cyclic modification
  Lys (10)..(10): Lys with a GLP-1 fusion 61 chemical modification
  Cys (29)..(29): Cys with a cyclic modification
  Arg (34)..(34): Arg with a N-Me chemical modification

SEQ ID NO: 258 - protein, 35 aa, Artificial Sequence; identical to SEQ ID NO: 20
  GLP-1 fusion coupled cyclic PYY peptide conjugate
  Ala (1)..(1): Ala, wherein the ala is a beta-alanine with a cyclic modification
  Lys (10)..(10): Lys with a GLP-1 fusion 63 chemical modification
  Cys (29)..(29): Cys with a cyclic modification
  Arg (34)..(34): Arg with a N-Me chemical modification

SEQ ID NO: 259 - protein, 35 aa, Artificial Sequence; identical to SEQ ID NO: 20
  GLP-1 fusion coupled cyclic PYY peptide conjugate
  Ala (1)..(1): Ala, wherein the ala is a beta-alanine with a cyclic modification
  Lys (10)..(10): Lys with a GLP-1 fusion 63 chemical modification
  Cys (29)..(29): Cys with a cyclic modification
  Arg (34)..(34): Arg with a psi-(R35, Y36) chemical modification
  Tyr (35)..(35): Tyr with a psi-(R35, Y36) chemical modification

SEQ ID NO: 260 - protein, 35 aa, Artificial Sequence; identical to SEQ ID NO: 20
  GLP-1 fusion coupled cyclic PYY peptide conjugate
  Ala (1)..(1): Ala, wherein the ala is a beta-alanine with a cyclic modification
  Lys (10)..(10): Lys with a GLP-1 fusion 40 chemical modification
  Cys (29)..(29): Cys with a cyclic modification
  Arg (34)..(34): Arg with a N-Me chemical modification

SEQ ID NO: 261 - protein, 35 aa, Artificial Sequence; identical to SEQ ID NO: 27
  GLP-1 fusion coupled cyclic PYY peptide conjugate
  Gly (1)..(1): Gly with a cyclic modification
  Lys (10)..(10): Lys with a GLP-1 fusion 40 chemical modification
  Cys (29)..(29): Cys with a cyclic modification
  Arg (34)..(34): Arg with a N-Me chemical modification

SEQ ID NO: 262 - protein, 35 aa, Artificial Sequence; identical to SEQ ID NO: 27
  GLP-1 fusion coupled cyclic PYY peptide conjugate
  Gly (1)..(1): Gly with a cyclic modification
  Lys (10)..(10): Lys with a GLP-1 fusion 34 chemical modification
  Cys (29)..(29): Cys with a cyclic modification
  Arg (34)..(34): Arg with a N-Me chemical modification

SEQ ID NO: 263 - protein, 20 aa, Artificial Sequence
  HGE for GLPD30
HGEGTFTSDVSSYLEEQAAK

SEQ ID NO: 264 - protein, 12 aa, Artificial Sequence
  HGE for GLPD31
HGEGTFTSDLSK

SEQ ID NO: 265 - protein, 16 aa, Artificial Sequence
  VVS peptide
VVSVLTVLHQDWLNGK

SEQ ID NO: 266 - protein, 6 aa, Artificial Sequence
  YYA peptide
YYASLR

SEQ ID NO: 267 - protein, 287 aa, Artificial Sequence
  GLP-1 fusion 113
HGEGTFTSDVSSYLEEQAAKEFIAWLVKGGGGGGGAGGGGAGGGGAAESKYGPPCPPCPAPEAAGGPSVFLFPPKPKDTLMISRTPEVTCVVVDVSQEDPEVQFNWYVDGVEVHNAKTKPREEQFNSTYRVVSVLTVLHQDWLNGKEYKCKVSNKGLPSSIEKTISKAKGQPREPQVYTLPPSQEEMTKNQVSLTCLVKGFYPSDIAVEWESNGQPENNYKTTPPVLDSDGSFFLYSRLTVDKSRWQEGNVFSCSVMHEALHNHYTQKSLSLSLGGGGGSGGGGSCA

SEQ ID NO: 268 - protein, 284 aa, Artificial Sequence
  GLP-1 fusion 114
HGEGTFTSDLSKQMEEEAVRLFIEWLKNGGGGAGGGGAGGGGAAESKYGPPCPPCPAPEAAGGPSVFLFPPKPKDTLMISRTPEVTCVVVDVSQEDPEVQFNWYVDGVEVHNAKTKPREEQFNSTYRVVSVLTVLHQDWLNGKEYKCKVSNKGLPSSIEKTISKAKGQPREPQVYTLPPSQEEMTKNQVSLTCLVKGFYPSDIAVEWESNGQPENNYKTTPPVLDSDGSFFLYSRLTVDKSRWQEGNVFSCSVMHEALHNHYTQKSLSLSLGGGGGSGGGGSCA

SEQ ID NO: 269 - protein, 293 aa, Artificial Sequence
  GLP-1 fusion 115
HGEGTFTSDVSSYLEEQAAKEFIAWLVKGGGGGGGAGGGGAGGGGAAESKYGPPCPPCPAPEAAGGPSVFLFPPKPKDTLMISRTPEVTCVVVDVSQEDPEVQFNWYVDGVEVHNAKTKPREEQFNSTYRVVSVLTVLHQDWLNGKEYKCKVSNKGLPSSIEKTISKAKGQPREPQVYTLPPSQEEMTKNQVSLTCLVKGFYPSDIAVEWESNGQPENNYKTTPPVLDSDGSFFLYSRLTVDKSRWQEGNVFSCSVMHEALHNHYTQKSLSLSLGGGGGSGGGGSGGGGGSCA

SEQ ID NO: 270 - protein, 290 aa, Artificial Sequence
  GLP-1 fusion 116
HGEGTFTSDLSKQMEEEAVRLFIEWLKNGGGGAGGGGAGGGGAAESKYGPPCPPCPAPEAAGGPSVFLFPPKPKDTLMISRTPEVTCVVVDVSQEDPEVQFNWYVDGVEVHNAKTKPREEQFNSTYRVVSVLTVLHQDWLNGKEYKCKVSNKGLPSSIEKTISKAKGQPREPQVYTLPPSQEEMTKNQVSLTCLVKGFYPSDIAVEWESNGQPENNYKTTPPVLDSDGSFFLYSRLTVDKSRWQEGNVFSCSVMHEALHNHYTQKSLSLSLGGGGGSGGGGSGGGGGSCA

SEQ ID NO: 271 - protein, 284 aa, Artificial Sequence
  GLP-1 fusion 117
HGEGTFTSDLSKQMEEEAVRLFIEWLKNGGGGSGGGGSGGGGSAESKYGPPCPPCPAPEAAGGPSVFLFPPKPKDTLMISRTPEVTCVVVDVSQEDPEVQFNWYVDGVEVHNAKTKPREEQFNSTYRVVSVLTVLHQDWLNGKEYKCKVSNKGLPSSIEKTISKAKGQPREPQVYTLPPSQEEMTKNQVSLTCLVKGFYPSDIAVEWESNGQPENNYKTTPPVLDSDGSFFLYSRLTVDKSRWQEGNVFSCSVMHEALHNHYTQKSLSLSLGGGGGSGGGGSCA

SEQ ID NO: 272 - protein, 295 aa, Artificial Sequence
  GLP-1 fusion 118
HGEGTFTSDLSKQMEEEAVRLFIEWLKNGGPSSGAPPPSGGGGSGGGGSGGGGSAESKYGPPCPPCPAPEAAGGPSVFLFPPKPKDTLMISRTPEVTCVVVDVSQEDPEVQFNWYVDGVEVHNAKTKPREEQFNSTYRVVSVLTVLHQDWLNGKEYKCKVSNKGLPSSIEKTISKAKGQPREPQVYTLPPSQEEMTKNQVSLTCLVKGFYPSDIAVEWESNGQPENNYKTTPPVLDSDGSFFLYSRLTVDKSRWQEGNVFSCSVMHEALHNHYTQKSLSLSLGGGGGSGGGGSCA

SEQ ID NO: 273 - protein, 289 aa, Artificial Sequence
  GLP-1 fusion 119
HGEGTFTSDLSKQMEEEAVRLFIEWLKNGGGGSGGGGSGGGGSAESKYGPPCPPCPAPEAAGGPSVFLFPPKPKDTLMISRTPEVTCVVVDVSQEDPEVQFNWYVDGVEVHNAKTKPREEQFNSTYRVVSVLTVLHQDWLNGKEYKCKVSNKGLPSSIEKTISKAKGQPREPQVYTLPPSQEEMTKNQVSLTCLVKGFYPSDIAVEWESNGQPENNYKTTPPVLDSDGSFFLYSRLTVDKSRWQEGNVFSCSVMHEALHNHYTQKSLSLSLGGGGGSGGGGSGGGGSCA

SEQ ID NO: 274 - protein, 300 aa, Artificial Sequence
  GLP-1 fusion 120
HGEGTFTSDLSKQMEEEAVRLFIEWLKNGGPSSGAPPPSGGGGSGGGGSGGGGSAESKYGPPCPPCPAPEAAGGPSVFLFPPKPKDTLMISRTPEVTCVVVDVSQEDPEVQFNWYVDGVEVHNAKTKPREEQFNSTYRVVSVLTVLHQDWLNGKEYKCKVSNKGLPSSIEKTISKAKGQPREPQVYTLPPSQEEMTKNQVSLTCLVKGFYPSDIAVEWESNGQPENNYKTTPPVLDSDGSFFLYSRLTVDKSRWQEGNVFSCSVMHEALHNHYTQKSLSLSLGGGGGSGGGGSGGGGSCA